European Patent Application EP 4 717 318 A2, published April 1, 2026. Title: ANTI-IL2 RECEPTOR GAMMA ANTIGEN-BINDING PROTEINS. Applicant: REGENERON PHARMACEUTICALS, INC. Application EP. The sequence listing filed with the application follows.

SEQUENCE LISTING (386 sequences)

SEQ ID NO: 1 - DNA, 369 bp, Homo sapiens
  source 1..369: mol_type = other DNA
caggtgcagctggtgcagtctggggctgaggtgaagaagcctggggcctcagtgcgggtctcctgcaaggcttctggatacaccttcaccgactacgatattcactgggtgcgacaggcccctggacatgggcttgagtggatggggtggatcaaccctaacagtggtggcacaaactatgcacagaagtttcagggcagggtcaccatgaccagggacacgtccatcagtacagtctacatggacctgagcaggctgagatctgacgacacggccgtgtattactgtgcgagagctgattatagtagttcgtattattattacggtatggacgtctggggccaagggaccacggtcaccgtctcctca

SEQ ID NO: 2 - protein, 123 aa, Homo sapiens
QVQLVQSGAEVKKPGASVRVSCKASGYTFTDYDIHWVRQAPGHGLEWMGWINPNSGGTNYAQKFQGRVTMTRDTSISTVYMDLSRLRSDDTAVYYCARADYSSSYYYYGMDVWGQGTTVTVSS

SEQ ID NO: 3 - DNA, 24 bp, Homo sapiens
  source 1..24: mol_type = other DNA
ggatacaccttcaccgactacgat

SEQ ID NO: 4 - protein, 8 aa, Homo sapiens
GYTFTDYD

SEQ ID NO: 5 - DNA, 24 bp, Homo sapiens
  source 1..24: mol_type = other DNA
atcaaccctaacagtggtggcaca

SEQ ID NO: 6 - protein, 8 aa, Homo sapiens
INPNSGGT

SEQ ID NO: 7 - DNA, 48 bp, Homo sapiens
  source 1..48: mol_type = other DNA
gcgagagctgattatagtagttcgtattattattacggtatggacgtc

SEQ ID NO: 8 - protein, 16 aa, Homo sapiens
ARADYSSSYYYYGMDV

SEQ ID NO: 9 - DNA, 339 bp, Homo sapiens
  source 1..339: mol_type = other DNA
gacatcgtgatgacccagtctccagactccctggctgtgtctctgggcgagagggccaccatcaactgcaagtccagccagagtgttttatacagctccaagaataagaactacttatcttggtaccagcagaaaccaggacagcctcctaagttgctcatttactgggcatctacccgggaattcggggtccctgaccgattcagtggccgcgggtctgggacagatttcactctcaccatcagcagcctgcaggctgaagatgtggcagtttattactgtcaacaatattatactactccgtacacttttggccaggggaccaagctggagatcaaa

SEQ ID NO: 10 - protein, 113 aa, Homo sapiens
DIVMTQSPDSLAVSLGERATINCKSSQSVLYSSKNKNYLSWYQQKPGQPPKLLIYWASTREFGVPDRFSGRGSGTDFTLTISSLQAEDVAVYYCQQYYTTPYTFGQGTKLEIK

SEQ ID NO: 11 - DNA, 36 bp, Homo sapiens
  source 1..36: mol_type = other DNA
cagagtgttttatacagctccaagaataagaactac

SEQ ID NO: 12 - protein, 12 aa, Homo sapiens
QSVLYSSKNKNY

SEQ ID NO: 13-14 - skipped (2 entries)

SEQ ID NO: 15 - DNA, 27 bp, Homo sapiens
  source 1..27: mol_type = other DNA
caacaatattatactactccgtacact

SEQ ID NO: 16 - protein, 9 aa, Homo sapiens
QQYYTTPYT

SEQ ID NO: 17 - DNA, 1353 bp, Homo sapiens
  source 1..1353: mol_type = other DNA
caggtgcagctggtgcagtctggggctgaggtgaagaagcctggggcctcagtgcgggtctcctgcaaggcttctggatacaccttcaccgactacgatattcactgggtgcgacaggcccctggacatgggcttgagtggatggggtggatcaaccctaacagtggtggcacaaactatgcacagaagtttcagggcagggtcaccatgaccagggacacgtccatcagtacagtctacatggacctgagcaggctgagatctgacgacacggccgtgtattactgtgcgagagctgattatagtagttcgtattattattacggtatggacgtctggggccaagggaccacggtcaccgtctcctcagcctccaccaagggcccatcggtcttccccctggcgccctgctccaggagcacctccgagagcacagccgccctgggctgcctggtcaaggactacttccccgaaccggtgacggtgtcgtggaactcaggcgccctgaccagcggcgtgcacaccttcccggctgtcctacagtcctcaggactctactccctcagcagcgtggtgaccgtgccctccagcagcttgggcacgaagacctacacctgcaacgtagatcacaagcccagcaacaccaaggtggacaagagagttgagtccaaatatggtcccccatgcccaccctgcccagcacctgagttcctggggggaccatcagtcttcctgttccccccaaaacccaaggacactctcatgatctcccggacccctgaggtcacgtgcgtggtggtggacgtgagccaggaagaccccgaggtccagttcaactggtacgtggatggcgtggaggtgcataatgccaagacaaagccgcgggaggagcagttcaacagcacgtaccgtgtggtcagcgtcctcaccgtcctgcaccaggactggctgaacggcaaggagtacaagtgcaaggtctccaacaaaggcctcccgtcctccatcgagaaaaccatctccaaagccaaagggcagccccgagagccacaggtgtacaccctgcccccatcccaggaggagatgaccaagaaccaggtcagcctgacctgcctggtcaaaggcttctaccccagcgacatcgccgtggagtgggagagcaatgggcagccggagaacaactacaagaccacgcctcccgtgctggactccgacggctccttcttcctctacagcaggctcaccgtggacaagagcaggtggcaggaggggaatgtcttctcatgctccgtgatgcatgaggctctgcacaaccactacacacagaagtccctctccctgtctctgggtaaatga

SEQ ID NO: 18 - protein, 450 aa, Homo sapiens
QVQLVQSGAEVKKPGASVRVSCKASGYTFTDYDIHWVRQAPGHGLEWMGWINPNSGGTNYAQKFQGRVTMTRDTSISTVYMDLSRLRSDDTAVYYCARADYSSSYYYYGMDVWGQGTTVTVSSASTKGPSVFPLAPCSRSTSESTAALGCLVKDYFPEPVTVSWNSGALTSGVHTFPAVLQSSGLYSLSSVVTVPSSSLGTKTYTCNVDHKPSNTKVDKRVESKYGPPCPPCPAPEFLGGPSVFLFPPKPKDTLMISRTPEVTCVVVDVSQEDPEVQFNWYVDGVEVHNAKTKPREEQFNSTYRVVSVLTVLHQDWLNGKEYKCKVSNKGLPSSIEKTISKAKGQPREPQVYTLPPSQEEMTKNQVSLTCLVKGFYPSDIAVEWESNGQPENNYKTTPPVLDSDGSFFLYSRLTVDKSRWQEGNVFSCSVMHEALHNHYTQKSLSLSLGK

SEQ ID NO: 19 - DNA, 663 bp, Homo sapiens
  source 1..663: mol_type = other DNA
gacatcgtgatgacccagtctccagactccctggctgtgtctctgggcgagagggccaccatcaactgcaagtccagccagagtgttttatacagctccaagaataagaactacttatcttggtaccagcagaaaccaggacagcctcctaagttgctcatttactgggcatctacccgggaattcggggtccctgaccgattcagtggccgcgggtctgggacagatttcactctcaccatcagcagcctgcaggctgaagatgtggcagtttattactgtcaacaatattatactactccgtacacttttggccaggggaccaagctggagatcaaacgaactgtggctgcaccatctgtcttcatcttcccgccatctgatgagcagttgaaatctggaactgcctctgttgtgtgcctgctgaataacttctatcccagagaggccaaagtacagtggaaggtggataacgccctccaatcgggtaactcccaggagagtgtcacagagcaggacagcaaggacagcacctacagcctcagcagcaccctgacgctgagcaaagcagactacgagaaacacaaagtctacgcctgcgaagtcacccatcagggcctgagctcgcccgtcacaaagagcttcaacaggggagagtgttag

SEQ ID NO: 20 - protein, 220 aa, Homo sapiens
DIVMTQSPDSLAVSLGERATINCKSSQSVLYSSKNKNYLSWYQQKPGQPPKLLIYWASTREFGVPDRFSGRGSGTDFTLTISSLQAEDVAVYYCQQYYTTPYTFGQGTKLEIKRTVAAPSVFIFPPSDEQLKSGTASVVCLLNNFYPREAKVQWKVDNALQSGNSQESVTEQDSKDSTYSLSSTLTLSKADYEKHKVYACEVTHQGLSSPVTKSFNRGEC

SEQ ID NO: 21 - DNA, 363 bp, Homo sapiens
  source 1..363: mol_type = other DNA
caggtgcagctggtggagtctgggggaggcgtggtccagcctgggaggtccctgagactctcctgtacagcctctggattcaccttcagaagttatgacatgtactgggtccgccaggctccaggcaaggggctggagtgggtgtcagttataacatatgatggaaataataaatactatgcagactccgtgaagggccgattcaccatctccagagacaattccaagaacacgctatttctgcaaatgagcagcctgagacctgaggacacggctgtttattactgtgcgaaaaggggcttaatatgggtcggggagtcctttgactactggggccagggaaccctggtcaccgtctcctca

SEQ ID NO: 22 - protein, 121 aa, Homo sapiens
QVQLVESGGGVVQPGRSLRLSCTASGFTFRSYDMYWVRQAPGKGLEWVSVITYDGNNKYYADSVKGRFTISRDNSKNTLFLQMSSLRPEDTAVYYCAKRGLIWVGESFDYWGQGTLVTVSS

SEQ ID NO: 23 - DNA, 24 bp, Homo sapiens
  source 1..24: mol_type = other DNA
ggattcaccttcagaagttatgac

SEQ ID NO: 24 - protein, 8 aa, Homo sapiens
GFTFRSYD

SEQ ID NO: 25 - DNA, 24 bp, Homo sapiens
  source 1..24: mol_type = other DNA
ataacatatgatggaaataataaa

SEQ ID NO: 26 - protein, 8 aa, Homo sapiens
ITYDGNNK

SEQ ID NO: 27 - DNA, 42 bp, Homo sapiens
  source 1..42: mol_type = other DNA
gcgaaaaggggcttaatatgggtcggggagtcctttgactac

SEQ ID NO: 28 - protein, 14 aa, Homo sapiens
AKRGLIWVGESFDY

SEQ ID NO: 29 - DNA, 321 bp, Homo sapiens
  source 1..321: mol_type = other DNA
gacatccagatgacccagtctccttccaccctgtctgcatctgtaggagacagagtcaccatcacttgccgggccagtcagagtattaatagctggttggcctggtatcagcagaaaccagggaaagcccctaacctcctgatctataaggcgtctagtttagaaagtggggtcccatcaaggttcagcggcagtggatctgggacagaattcactctcaccatcagcagcctgcagcctgatgattttgcaacttattactgccaacagtataagagttattcgtggacgttcggccaagggaccaaggtggaaatcaaa

SEQ ID NO: 30 - protein, 107 aa, Homo sapiens
DIQMTQSPSTLSASVGDRVTITCRASQSINSWLAWYQQKPGKAPNLLIYKASSLESGVPSRFSGSGSGTEFTLTISSLQPDDFATYYCQQYKSYSWTFGQGTKVEIK

SEQ ID NO: 31 - DNA, 18 bp, Homo sapiens
  source 1..18: mol_type = other DNA
cagagtattaatagctgg

SEQ ID NO: 32 - protein, 6 aa, Homo sapiens
QSINSW

SEQ ID NO: 33-34 - skipped (2 entries)

SEQ ID NO: 35 - DNA, 27 bp, Homo sapiens
  source 1..27: mol_type = other DNA
caacagtataagagttattcgtggacg

SEQ ID NO: 36 - protein, 9 aa, Homo sapiens
QQYKSYSWT

SEQ ID NO: 37 - DNA, 1347 bp, Homo sapiens
  source 1..1347: mol_type = other DNA
caggtgcagctggtggagtctgggggaggcgtggtccagcctgggaggtccctgagactctcctgtacagcctctggattcaccttcagaagttatgacatgtactgggtccgccaggctccaggcaaggggctggagtgggtgtcagttataacatatgatggaaataataaatactatgcagactccgtgaagggccgattcaccatctccagagacaattccaagaacacgctatttctgcaaatgagcagcctgagacctgaggacacggctgtttattactgtgcgaaaaggggcttaatatgggtcggggagtcctttgactactggggccagggaaccctggtcaccgtctcctcagcctccaccaagggcccatcggtcttccccctggcgccctgctccaggagcacctccgagagcacagccgccctgggctgcctggtcaaggactacttccccgaaccggtgacggtgtcgtggaactcaggcgccctgaccagcggcgtgcacaccttcccggctgtcctacagtcctcaggactctactccctcagcagcgtggtgaccgtgccctccagcagcttgggcacgaagacctacacctgcaacgtagatcacaagcccagcaacaccaaggtggacaagagagttgagtccaaatatggtcccccatgcccaccctgcccagcacctgagttcctggggggaccatcagtcttcctgttccccccaaaacccaaggacactctcatgatctcccggacccctgaggtcacgtgcgtggtggtggacgtgagccaggaagaccccgaggtccagttcaactggtacgtggatggcgtggaggtgcataatgccaagacaaagccgcgggaggagcagttcaacagcacgtaccgtgtggtcagcgtcctcaccgtcctgcaccaggactggctgaacggcaaggagtacaagtgcaaggtctccaacaaaggcctcccgtcctccatcgagaaaaccatctccaaagccaaagggcagccccgagagccacaggtgtacaccctgcccccatcccaggaggagatgaccaagaaccaggtcagcctgacctgcctggtcaaaggcttctaccccagcgacatcgccgtggagtgggagagcaatgggcagccggagaacaactacaagaccacgcctcccgtgctggactccgacggctccttcttcctctacagcaggctcaccgtggacaagagcaggtggcaggaggggaatgtcttctcatgctccgtgatgcatgaggctctgcacaaccactacacacagaagtccctctccctgtctctgggtaaatga

SEQ ID NO: 38 - protein, 448 aa, Homo sapiens
QVQLVESGGGVVQPGRSLRLSCTASGFTFRSYDMYWVRQAPGKGLEWVSVITYDGNNKYYADSVKGRFTISRDNSKNTLFLQMSSLRPEDTAVYYCAKRGLIWVGESFDYWGQGTLVTVSSASTKGPSVFPLAPCSRSTSESTAALGCLVKDYFPEPVTVSWNSGALTSGVHTFPAVLQSSGLYSLSSVVTVPSSSLGTKTYTCNVDHKPSNTKVDKRVESKYGPPCPPCPAPEFLGGPSVFLFPPKPKDTLMISRTPEVTCVVVDVSQEDPEVQFNWYVDGVEVHNAKTKPREEQFNSTYRVVSVLTVLHQDWLNGKEYKCKVSNKGLPSSIEKTISKAKGQPREPQVYTLPPSQEEMTKNQVSLTCLVKGFYPSDIAVEWESNGQPENNYKTTPPVLDSDGSFFLYSRLTVDKSRWQEGNVFSCSVMHEALHNHYTQKSLSLSLGK

SEQ ID NO: 39 - DNA, 645 bp, Homo sapiens
  source 1..645: mol_type = other DNA
gacatccagatgacccagtctccttccaccctgtctgcatctgtaggagacagagtcaccatcacttgccgggccagtcagagtattaatagctggttggcctggtatcagcagaaaccagggaaagcccctaacctcctgatctataaggcgtctagtttagaaagtggggtcccatcaaggttcagcggcagtggatctgggacagaattcactctcaccatcagcagcctgcagcctgatgattttgcaacttattactgccaacagtataagagttattcgtggacgttcggccaagggaccaaggtggaaatcaaacgaactgtggctgcaccatctgtcttcatcttcccgccatctgatgagcagttgaaatctggaactgcctctgttgtgtgcctgctgaataacttctatcccagagaggccaaagtacagtggaaggtggataacgccctccaatcgggtaactcccaggagagtgtcacagagcaggacagcaaggacagcacctacagcctcagcagcaccctgacgctgagcaaagcagactacgagaaacacaaagtctacgcctgcgaagtcacccatcagggcctgagctcgcccgtcacaaagagcttcaacaggggagagtgttag

SEQ ID NO: 40 - protein, 214 aa, Homo sapiens
DIQMTQSPSTLSASVGDRVTITCRASQSINSWLAWYQQKPGKAPNLLIYKASSLESGVPSRFSGSGSGTEFTLTISSLQPDDFATYYCQQYKSYSWTFGQGTKVEIKRTVAAPSVFIFPPSDEQLKSGTASVVCLLNNFYPREAKVQWKVDNALQSGNSQESVTEQDSKDSTYSLSSTLTLSKADYEKHKVYACEVTHQGLSSPVTKSFNRGEC

SEQ ID NO: 41 - DNA, 360 bp, Homo sapiens
  source 1..360: mol_type = other DNA
caggtgcagctggtggagtctgggggaggcgtggtccagcctgggaggtccctgagactctcctgtgcagcctctggattcaacttcagaaactttggcatgcactgggtccgccaggctccaggcaaggggctggaatgggtggcaggtatattatatgatggaagtagtaaatactatgcagactccgtgaaggaccgattcaccatctccagagacaattccaagaacacgctgtttctgcaaatgaacagcctgagagctgaggacacggctatgtattactgtgcgaaagaggaggacacagccatggttccttttgattcctggggcccgggaaccctggtcaccgtctcctca

SEQ ID NO: 42 - protein, 120 aa, Homo sapiens
QVQLVESGGGVVQPGRSLRLSCAASGFNFRNFGMHWVRQAPGKGLEWVAGILYDGSSKYYADSVKDRFTISRDNSKNTLFLQMNSLRAEDTAMYYCAKEEDTAMVPFDSWGPGTLVTVSS

SEQ ID NO: 43 - DNA, 24 bp, Homo sapiens
  source 1..24: mol_type = other DNA
ggattcaacttcagaaactttggc

SEQ ID NO: 44 - protein, 8 aa, Homo sapiens
GFNFRNFG

SEQ ID NO: 45 - DNA, 24 bp, Homo sapiens
  source 1..24: mol_type = other DNA
atattatatgatggaagtagtaaa

SEQ ID NO: 46 - protein, 8 aa, Homo sapiens
ILYDGSSK

SEQ ID NO: 47 - DNA, 39 bp, Homo sapiens
  source 1..39: mol_type = other DNA
gcgaaagaggaggacacagccatggttccttttgattcc

SEQ ID NO: 48 - protein, 13 aa, Homo sapiens
AKEEDTAMVPFDS

SEQ ID NO: 49 - DNA, 321 bp, Homo sapiens
  source 1..321: mol_type = other DNA
gacatccagttgacccagtctccatccttcctgtctgcttctgtaggagacagagtcaccatcacttgctgggccagtcagggcattagtagttatttagcctggtatcagcaaaaaccagggaaagcccctaccctcctgatctatgctgcgtccactttgcaaagtggggtcccatcaaggttcagcggcagtggatctgggacagaattcactctcacaatcagcagcctgcagcctgaagattttgcaagttattactgtcaacagcttaagagttacccgctcactttcggcggagggaccaaggtggagatcaaa

SEQ ID NO: 50 - protein, 107 aa, Homo sapiens
DIQLTQSPSFLSASVGDRVTITCWASQGISSYLAWYQQKPGKAPTLLIYAASTLQSGVPSRFSGSGSGTEFTLTISSLQPEDFASYYCQQLKSYPLTFGGGTKVEIK

SEQ ID NO: 51 - DNA, 18 bp, Homo sapiens
  source 1..18: mol_type = other DNA
cagggcattagtagttat

SEQ ID NO: 52 - protein, 6 aa, Homo sapiens
QGISSY

SEQ ID NO: 53-54 - skipped (2 entries)

SEQ ID NO: 55 - DNA, 27 bp, Homo sapiens
  source 1..27: mol_type = other DNA
caacagcttaagagttacccgctcact

SEQ ID NO: 56 - protein, 9 aa, Homo sapiens
QQLKSYPLT

SEQ ID NO: 57 - DNA, 1344 bp, Homo sapiens
  source 1..1344: mol_type = other DNA
caggtgcagctggtggagtctgggggaggcgtggtccagcctgggaggtccctgagactctcctgtgcagcctctggattcaacttcagaaactttggcatgcactgggtccgccaggctccaggcaaggggctggaatgggtggcaggtatattatatgatggaagtagtaaatactatgcagactccgtgaaggaccgattcaccatctccagagacaattccaagaacacgctgtttctgcaaatgaacagcctgagagctgaggacacggctatgtattactgtgcgaaagaggaggacacagccatggttccttttgattcctggggcccgggaaccctggtcaccgtctcctcagcctccaccaagggcccatcggtcttccccctggcgccctgctccaggagcacctccgagagcacagccgccctgggctgcctggtcaaggactacttccccgaaccggtgacggtgtcgtggaactcaggcgccctgaccagcggcgtgcacaccttcccggctgtcctacagtcctcaggactctactccctcagcagcgtggtgaccgtgccctccagcagcttgggcacgaagacctacacctgcaacgtagatcacaagcccagcaacaccaaggtggacaagagagttgagtccaaatatggtcccccatgcccaccctgcccagcacctgagttcctggggggaccatcagtcttcctgttccccccaaaacccaaggacactctcatgatctcccggacccctgaggtcacgtgcgtggtggtggacgtgagccaggaagaccccgaggtccagttcaactggtacgtggatggcgtggaggtgcataatgccaagacaaagccgcgggaggagcagttcaacagcacgtaccgtgtggtcagcgtcctcaccgtcctgcaccaggactggctgaacggcaaggagtacaagtgcaaggtctccaacaaaggcctcccgtcctccatcgagaaaaccatctccaaagccaaagggcagccccgagagccacaggtgtacaccctgcccccatcccaggaggagatgaccaagaaccaggtcagcctgacctgcctggtcaaaggcttctaccccagcgacatcgccgtggagtgggagagcaatgggcagccggagaacaactacaagaccacgcctcccgtgctggactccgacggctccttcttcctctacagcaggctcaccgtggacaagagcaggtggcaggaggggaatgtcttctcatgctccgtgatgcatgaggctctgcacaaccactacacacagaagtccctctccctgtctctgggtaaatga

SEQ ID NO: 58 - protein, 447 aa, Homo sapiens
QVQLVESGGGVVQPGRSLRLSCAASGFNFRNFGMHWVRQAPGKGLEWVAGILYDGSSKYYADSVKDRFTISRDNSKNTLFLQMNSLRAEDTAMYYCAKEEDTAMVPFDSWGPGTLVTVSSASTKGPSVFPLAPCSRSTSESTAALGCLVKDYFPEPVTVSWNSGALTSGVHTFPAVLQSSGLYSLSSVVTVPSSSLGTKTYTCNVDHKPSNTKVDKRVESKYGPPCPPCPAPEFLGGPSVFLFPPKPKDTLMISRTPEVTCVVVDVSQEDPEVQFNWYVDGVEVHNAKTKPREEQFNSTYRVVSVLTVLHQDWLNGKEYKCKVSNKGLPSSIEKTISKAKGQPREPQVYTLPPSQEEMTKNQVSLTCLVKGFYPSDIAVEWESNGQPENNYKTTPPVLDSDGSFFLYSRLTVDKSRWQEGNVFSCSVMHEALHNHYTQKSLSLSLGK

SEQ ID NO: 59 - DNA, 645 bp, Homo sapiens
  source 1..645: mol_type = other DNA
gacatccagttgacccagtctccatccttcctgtctgcttctgtaggagacagagtcaccatcacttgctgggccagtcagggcattagtagttatttagcctggtatcagcaaaaaccagggaaagcccctaccctcctgatctatgctgcgtccactttgcaaagtggggtcccatcaaggttcagcggcagtggatctgggacagaattcactctcacaatcagcagcctgcagcctgaagattttgcaagttattactgtcaacagcttaagagttacccgctcactttcggcggagggaccaaggtggagatcaaacgaactgtggctgcaccatctgtcttcatcttcccgccatctgatgagcagttgaaatctggaactgcctctgttgtgtgcctgctgaataacttctatcccagagaggccaaagtacagtggaaggtggataacgccctccaatcgggtaactcccaggagagtgtcacagagcaggacagcaaggacagcacctacagcctcagcagcaccctgacgctgagcaaagcagactacgagaaacacaaagtctacgcctgcgaagtcacccatcagggcctgagctcgcccgtcacaaagagcttcaacaggggagagtgttag

SEQ ID NO: 60 - protein, 214 aa, Homo sapiens
DIQLTQSPSFLSASVGDRVTITCWASQGISSYLAWYQQKPGKAPTLLIYAASTLQSGVPSRFSGSGSGTEFTLTISSLQPEDFASYYCQQLKSYPLTFGGGTKVEIKRTVAAPSVFIFPPSDEQLKSGTASVVCLLNNFYPREAKVQWKVDNALQSGNSQESVTEQDSKDSTYSLSSTLTLSKADYEKHKVYACEVTHQGLSSPVTKSFNRGEC

SEQ ID NO: 61 - DNA, 366 bp, Homo sapiens
  source 1..366: mol_type = other DNA
caggtgcagctgcaggagtcgggcccaggactggtgaagccttcacagaccctgtccctcacctgcactgtctctggtggctccatcagcagtggtggttactactggagctggatccgccagcacccagggaagggcctggagtggattggtttcatctattacagtgggaagacctactacaacccgtccctcaagagtcgacttaccatctcagtagacacgtctaagagccagttctccctgaagctgaggtctgtgactgccgcggacacggccgtgtattactgtgcgagactggggtataccaactcggccgggtggttcgacccctggggccagggaaccctggtcaccgtctcctca

SEQ ID NO: 62 - protein, 122 aa, Homo sapiens
QVQLQESGPGLVKPSQTLSLTCTVSGGSISSGGYYWSWIRQHPGKGLEWIGFIYYSGKTYYNPSLKSRLTISVDTSKSQFSLKLRSVTAADTAVYYCARLGYTNSAGWFDPWGQGTLVTVSS

SEQ ID NO: 63 - DNA, 30 bp, Homo sapiens
  source 1..30: mol_type = other DNA
ggtggctccatcagcagtggtggttactac

SEQ ID NO: 64 - protein, 10 aa, Homo sapiens
GGSISSGGYY

SEQ ID NO: 65 - DNA, 21 bp, Homo sapiens
  source 1..21: mol_type = other DNA
atctattacagtgggaagacc

SEQ ID NO: 66 - protein, 7 aa, Homo sapiens
IYYSGKT

SEQ ID NO: 67 - DNA, 42 bp, Homo sapiens
  source 1..42: mol_type = other DNA
gcgagactggggtataccaactcggccgggtggttcgacccc

SEQ ID NO: 68 - protein, 14 aa, Homo sapiens
ARLGYTNSAGWFDP

SEQ ID NO: 69 - DNA, 321 bp, Homo sapiens
  source 1..321: mol_type = other DNA
gacatccagatgacccagtctccatcctccctgtctgcatctgtaggagacagagtcaccatcacttgccgggcaagtcagagcattagcagctatttaaattggtatcagcagaaaccagggaaagcccctaacctcctgatctatgctgcatccagtttgcaaagtggggtcccatcaaggttcagtggcagtggatctgggacagatttcactctcaccatcagcagtctgcaacctgaagatcttgcaacttactactgtcaacagagttacacaaccccattcactttcggccctgggaccaaagtggatatcaaa

SEQ ID NO: 70 - protein, 107 aa, Homo sapiens
DIQMTQSPSSLSASVGDRVTITCRASQSISSYLNWYQQKPGKAPNLLIYAASSLQSGVPSRFSGSGSGTDFTLTISSLQPEDLATYYCQQSYTTPFTFGPGTKVDIK

SEQ ID NO: 71 - DNA, 18 bp, Homo sapiens
  source 1..18: mol_type = other DNA
cagagcattagcagctat

SEQ ID NO: 72 - protein, 6 aa, Homo sapiens
QSISSY

SEQ ID NO: 73 - skipped

SEQ ID NO: 74 - DNA, 27 bp, Homo sapiens
  source 1..27: mol_type = other DNA
caacagagttacacaaccccattcact

SEQ ID NO: 75 - protein, 9 aa, Homo sapiens
QQSYTTPFT

SEQ ID NO: 76 - DNA, 1350 bp, Homo sapiens
  source 1..1350: mol_type = other DNA
caggtgcagctgcaggagtcgggcccaggactggtgaagccttcacagaccctgtccctcacctgcactgtctctggtggctccatcagcagtggtggttactactggagctggatccgccagcacccagggaagggcctggagtggattggtttcatctattacagtgggaagacctactacaacccgtccctcaagagtcgacttaccatctcagtagacacgtctaagagccagttctccctgaagctgaggtctgtgactgccgcggacacggccgtgtattactgtgcgagactggggtataccaactcggccgggtggttcgacccctggggccagggaaccctggtcaccgtctcctcagcctccaccaagggcccatcggtcttccccctggcgccctgctccaggagcacctccgagagcacagccgccctgggctgcctggtcaaggactacttccccgaaccggtgacggtgtcgtggaactcaggcgccctgaccagcggcgtgcacaccttcccggctgtcctacagtcctcaggactctactccctcagcagcgtggtgaccgtgccctccagcagcttgggcacgaagacctacacctgcaacgtagatcacaagcccagcaacaccaaggtggacaagagagttgagtccaaatatggtcccccatgcccaccctgcccagcacctgagttcctggggggaccatcagtcttcctgttccccccaaaacccaaggacactctcatgatctcccggacccctgaggtcacgtgcgtggtggtggacgtgagccaggaagaccccgaggtccagttcaactggtacgtggatggcgtggaggtgcataatgccaagacaaagccgcgggaggagcagttcaacagcacgtaccgtgtggtcagcgtcctcaccgtcctgcaccaggactggctgaacggcaaggagtacaagtgcaaggtctccaacaaaggcctcccgtcctccatcgagaaaaccatctccaaagccaaagggcagccccgagagccacaggtgtacaccctgcccccatcccaggaggagatgaccaagaaccaggtcagcctgacctgcctggtcaaaggcttctaccccagcgacatcgccgtggagtgggagagcaatgggcagccggagaacaactacaagaccacgcctcccgtgctggactccgacggctccttcttcctctacagcaggctcaccgtggacaagagcaggtggcaggaggggaatgtcttctcatgctccgtgatgcatgaggctctgcacaaccactacacacagaagtccctctccctgtctctgggtaaatga

SEQ ID NO: 77 - protein, 449 aa, Homo sapiens
QVQLQESGPGLVKPSQTLSLTCTVSGGSISSGGYYWSWIRQHPGKGLEWIGFIYYSGKTYYNPSLKSRLTISVDTSKSQFSLKLRSVTAADTAVYYCARLGYTNSAGWFDPWGQGTLVTVSSASTKGPSVFPLAPCSRSTSESTAALGCLVKDYFPEPVTVSWNSGALTSGVHTFPAVLQSSGLYSLSSVVTVPSSSLGTKTYTCNVDHKPSNTKVDKRVESKYGPPCPPCPAPEFLGGPSVFLFPPKPKDTLMISRTPEVTCVVVDVSQEDPEVQFNWYVDGVEVHNAKTKPREEQFNSTYRVVSVLTVLHQDWLNGKEYKCKVSNKGLPSSIEKTISKAKGQPREPQVYTLPPSQEEMTKNQVSLTCLVKGFYPSDIAVEWESNGQPENNYKTTPPVLDSDGSFFLYSRLTVDKSRWQEGNVFSCSVMHEALHNHYTQKSLSLSLGK

SEQ ID NO: 78 - DNA, 645 bp, Homo sapiens
  source 1..645: mol_type = other DNA
gacatccagatgacccagtctccatcctccctgtctgcatctgtaggagacagagtcaccatcacttgccgggcaagtcagagcattagcagctatttaaattggtatcagcagaaaccagggaaagcccctaacctcctgatctatgctgcatccagtttgcaaagtggggtcccatcaaggttcagtggcagtggatctgggacagatttcactctcaccatcagcagtctgcaacctgaagatcttgcaacttactactgtcaacagagttacacaaccccattcactttcggccctgggaccaaagtggatatcaaacgaactgtggctgcaccatctgtcttcatcttcccgccatctgatgagcagttgaaatctggaactgcctctgttgtgtgcctgctgaataacttctatcccagagaggccaaagtacagtggaaggtggataacgccctccaatcgggtaactcccaggagagtgtcacagagcaggacagcaaggacagcacctacagcctcagcagcaccctgacgctgagcaaagcagactacgagaaacacaaagtctacgcctgcgaagtcacccatcagggcctgagctcgcccgtcacaaagagcttcaacaggggagagtgttag

SEQ ID NO: 79 - protein, 214 aa, Homo sapiens
DIQMTQSPSSLSASVGDRVTITCRASQSISSYLNWYQQKPGKAPNLLIYAASSLQSGVPSRFSGSGSGTDFTLTISSLQPEDLATYYCQQSYTTPFTFGPGTKVDIKRTVAAPSVFIFPPSDEQLKSGTASVVCLLNNFYPREAKVQWKVDNALQSGNSQESVTEQDSKDSTYSLSSTLTLSKADYEKHKVYACEVTHQGLSSPVTKSFNRGEC

SEQ ID NO: 80 - DNA, 375 bp, Homo sapiens
  source 1..375: mol_type = other DNA
gaggtgcagctggtggagtcggggggaggtttggtaaagcctggggggtcccttagactctcctgtgcagcctctggattcactttcagtaccgcctggatgagctgggtccgccagtctccagggagggggctggagtgggttggccgtatgaaaagcaagactgatggtgggacaacattctacgctgcacccgtgaaaggcagattcaccatctcaagagatgattcaaaaaacacactgtatctgcaaatgaacagcctgaaaaccgaggacacagccgtttattactgtaccacaggattagtcccggccttctataagtactacggcgtggacgtctggggccaagggaccacggtcaccgtctcctca

SEQ ID NO: 81 - protein, 125 aa, Homo sapiens
EVQLVESGGGLVKPGGSLRLSCAASGFTFSTAWMSWVRQSPGRGLEWVGRMKSKTDGGTTFYAAPVKGRFTISRDDSKNTLYLQMNSLKTEDTAVYYCTTGLVPAFYKYYGVDVWGQGTTVTVSS

SEQ ID NO: 82 - DNA, 24 bp, Homo sapiens
  source 1..24: mol_type = other DNA
ggattcactttcagtaccgcctgg

SEQ ID NO: 83 - protein, 8 aa, Homo sapiens
GFTFSTAW

SEQ ID NO: 84 - DNA, 30 bp, Homo sapiens
  source 1..30: mol_type = other DNA
atgaaaagcaagactgatggtgggacaaca

SEQ ID NO: 85 - protein, 10 aa, Homo sapiens
MKSKTDGGTT

SEQ ID NO: 86 - DNA, 48 bp, Homo sapiens
  source 1..48: mol_type = other DNA
accacaggattagtcccggccttctataagtactacggcgtggacgtc

SEQ ID NO: 87 - protein, 16 aa, Homo sapiens
TTGLVPAFYKYYGVDV

SEQ ID NO: 88 - DNA, 318 bp, Homo sapiens
  source 1..318: mol_type = other DNA
gacatccagatgacccagtctccatcctccctgtctgcatctgtaggagacagaatcaccatcacttgccaggcgagtcaggacattaccaactatttaaattggtatcagcagaagccagggaaagcccctaacctcctgatctacgatgcatccaatttggttacaggggtcccatcaaggttcagtggaagtggatctgggacagattttactttcaccatcctcagcctgcagcctgaagatattgcaacatattactgtcaacagtatgatagtctcctcactttcggccctgggaccaaagtggatatcaaa

SEQ ID NO: 89 - protein, 106 aa, Homo sapiens
DIQMTQSPSSLSASVGDRITITCQASQDITNYLNWYQQKPGKAPNLLIYDASNLVTGVPSRFSGSGSGTDFTFTILSLQPEDIATYYCQQYDSLLTFGPGTKVDIK

SEQ ID NO: 90 - DNA, 18 bp, Homo sapiens
  source 1..18: mol_type = other DNA
caggacattaccaactat

SEQ ID NO: 91 - protein, 6 aa, Homo sapiens
QDITNY

SEQ ID NO: 92-93 - skipped (2 entries)

SEQ ID NO: 94 - DNA, 24 bp, Homo sapiens
  source 1..24: mol_type = other DNA
caacagtatgatagtctcctcact

SEQ ID NO: 95 - protein, 8 aa, Homo sapiens
QQYDSLLT

SEQ ID NO: 96 - DNA, 1359 bp, Homo sapiens
  source 1..1359: mol_type = other DNA
gaggtgcagctggtggagtcggggggaggtttggtaaagcctggggggtcccttagactctcctgtgcagcctctggattcactttcagtaccgcctggatgagctgggtccgccagtctccagggagggggctggagtgggttggccgtatgaaaagcaagactgatggtgggacaacattctacgctgcacccgtgaaaggcagattcaccatctcaagagatgattcaaaaaacacactgtatctgcaaatgaacagcctgaaaaccgaggacacagccgtttattactgtaccacaggattagtcccggccttctataagtactacggcgtggacgtctggggccaagggaccacggtcaccgtctcctcagcctccaccaagggcccatcggtcttccccctggcgccctgctccaggagcacctccgagagcacagccgccctgggctgcctggtcaaggactacttccccgaaccggtgacggtgtcgtggaactcaggcgccctgaccagcggcgtgcacaccttcccggctgtcctacagtcctcaggactctactccctcagcagcgtggtgaccgtgccctccagcagcttgggcacgaagacctacacctgcaacgtagatcacaagcccagcaacaccaaggtggacaagagagttgagtccaaatatggtcccccatgcccaccctgcccagcacctgagttcctggggggaccatcagtcttcctgttccccccaaaacccaaggacactctcatgatctcccggacccctgaggtcacgtgcgtggtggtggacgtgagccaggaagaccccgaggtccagttcaactggtacgtggatggcgtggaggtgcataatgccaagacaaagccgcgggaggagcagttcaacagcacgtaccgtgtggtcagcgtcctcaccgtcctgcaccaggactggctgaacggcaaggagtacaagtgcaaggtctccaacaaaggcctcccgtcctccatcgagaaaaccatctccaaagccaaagggcagccccgagagccacaggtgtacaccctgcccccatcccaggaggagatgaccaagaaccaggtcagcctgacctgcctggtcaaaggcttctaccccagcgacatcgccgtggagtgggagagcaatgggcagccggagaacaactacaagaccacgcctcccgtgctggactccgacggctccttcttcctctacagcaggctcaccgtggacaagagcaggtggcaggaggggaatgtcttctcatgctccgtgatgcatgaggctctgcacaaccactacacacagaagtccctctccctgtctctgggtaaatga

SEQ ID NO: 97 - protein, 452 aa, Homo sapiens
EVQLVESGGGLVKPGGSLRLSCAASGFTFSTAWMSWVRQSPGRGLEWVGRMKSKTDGGTTFYAAPVKGRFTISRDDSKNTLYLQMNSLKTEDTAVYYCTTGLVPAFYKYYGVDVWGQGTTVTVSSASTKGPSVFPLAPCSRSTSESTAALGCLVKDYFPEPVTVSWNSGALTSGVHTFPAVLQSSGLYSLSSVVTVPSSSLGTKTYTCNVDHKPSNTKVDKRVESKYGPPCPPCPAPEFLGGPSVFLFPPKPKDTLMISRTPEVTCVVVDVSQEDPEVQFNWYVDGVEVHNAKTKPREEQFNSTYRVVSVLTVLHQDWLNGKEYKCKVSNKGLPSSIEKTISKAKGQPREPQVYTLPPSQEEMTKNQVSLTCLVKGFYPSDIAVEWESNGQPENNYKTTPPVLDSDGSFFLYSRLTVDKSRWQEGNVFSCSVMHEALHNHYTQKSLSLSLGK

SEQ ID NO: 98 - DNA, 642 bp, Homo sapiens
  source 1..642: mol_type = other DNA
gacatccagatgacccagtctccatcctccctgtctgcatctgtaggagacagaatcaccatcacttgccaggcgagtcaggacattaccaactatttaaattggtatcagcagaagccagggaaagcccctaacctcctgatctacgatgcatccaatttggttacaggggtcccatcaaggttcagtggaagtggatctgggacagattttactttcaccatcctcagcctgcagcctgaagatattgcaacatattactgtcaacagtatgatagtctcctcactttcggccctgggaccaaagtggatatcaaacgaactgtggctgcaccatctgtcttcatcttcccgccatctgatgagcagttgaaatctggaactgcctctgttgtgtgcctgctgaataacttctatcccagagaggccaaagtacagtggaaggtggataacgccctccaatcgggtaactcccaggagagtgtcacagagcaggacagcaaggacagcacctacagcctcagcagcaccctgacgctgagcaaagcagactacgagaaacacaaagtctacgcctgcgaagtcacccatcagggcctgagctcgcccgtcacaaagagcttcaacaggggagagtgttag

SEQ ID NO: 99 - protein, 213 aa, Homo sapiens
DIQMTQSPSSLSASVGDRITITCQASQDITNYLNWYQQKPGKAPNLLIYDASNLVTGVPSRFSGSGSGTDFTFTILSLQPEDIATYYCQQYDSLLTFGPGTKVDIKRTVAAPSVFIFPPSDEQLKSGTASVVCLLNNFYPREAKVQWKVDNALQSGNSQESVTEQDSKDSTYSLSSTLTLSKADYEKHKVYACEVTHQGLSSPVTKSFNRGEC

SEQ ID NO: 100 - DNA, 369 bp, Homo sapiens
  source 1..369: mol_type = other DNA
gaggtgcagctggtggagtctgggggaggcttggtccagcctggggggtccctgagactctcctgtgcagcctctggattcaccttcaataactatgcaatgcactgggtccgccaggctcccgggaagggactggaatatgtttcatctattagtagtagtgggggtagcacatattatgaagactctgtgaagggcagattcaccatctccagagacaattccaagaacacgctgtatcttcaaatgggcagcctgagagctgaggacatggctgtgtattactgtgcgagatcattctatggttcggggacttattatgatacttttgatatgtggggccaagggacaatggtcaccgtctcttca

SEQ ID NO: 101 - protein, 123 aa, Homo sapiens
EVQLVESGGGLVQPGGSLRLSCAASGFTFNNYAMHWVRQAPGKGLEYVSSISSSGGSTYYEDSVKGRFTISRDNSKNTLYLQMGSLRAEDMAVYYCARSFYGSGTYYDTFDMWGQGTMVTVSS

SEQ ID NO: 102 - DNA, 24 bp, Homo sapiens
  source 1..24: mol_type = other DNA
ggattcaccttcaataactatgca

SEQ ID NO: 103 - protein, 8 aa, Homo sapiens
GFTFNNYA

SEQ ID NO: 104 - DNA, 24 bp, Homo sapiens
  source 1..24: mol_type = other DNA
attagtagtagtgggggtagcaca

SEQ ID NO: 105 - protein, 8 aa, Homo sapiens
ISSSGGST

SEQ ID NO: 106 - DNA, 48 bp, Homo sapiens
  source 1..48: mol_type = other DNA
gcgagatcattctatggttcggggacttattatgatacttttgatatg

SEQ ID NO: 107 - protein, 16 aa, Homo sapiens
ARSFYGSGTYYDTFDM

SEQ ID NO: 108 - DNA, 321 bp, Homo sapiens
  source 1..321: mol_type = other DNA
gacatccagatgacccagtctccatcctccctgtctgcatctataggagacagagtcaccatcacttgccgggcaagtcagagcattagcaggtatttaaattggtatcagcagaaaccagggaaagcccctaagctcctgatctatgctgcatccagtttgcaaagtggggtcccatcaaggttcagtgccagtggatctgggacagatttcactctcaccatcagcagtctgcaacctgaagattttgcaacttactactgtcaacagagttacagtaccccgttcacttttggccaggggaccaagctggagatcaaa

SEQ ID NO: 109 - protein, 107 aa, Homo sapiens
DIQMTQSPSSLSASIGDRVTITCRASQSISRYLNWYQQKPGKAPKLLIYAASSLQSGVPSRFSASGSGTDFTLTISSLQPEDFATYYCQQSYSTPFTFGQGTKLEIK

SEQ ID NO: 110 - DNA, 18 bp, Homo sapiens
  source 1..18: mol_type = other DNA
cagagcattagcaggtat

SEQ ID NO: 111 - protein, 6 aa, Homo sapiens
QSISRY

SEQ ID NO: 112 - DNA, 27 bp, Homo sapiens
  source 1..27: mol_type = other DNA
caacagagttacagtaccccgttcact

SEQ ID NO: 113 - protein, 9 aa, Homo sapiens
QQSYSTPFT

SEQ ID NO: 114 - DNA, 1353 bp, Homo sapiens
  source 1..1353: mol_type = other DNA
gaggtgcagctggtggagtctgggggaggcttggtccagcctggggggtccctgagactctcctgtgcagcctctggattcaccttcaataactatgcaatgcactgggtccgccaggctcccgggaagggactggaatatgtttcatctattagtagtagtgggggtagcacatattatgaagactctgtgaagggcagattcaccatctccagagacaattccaagaacacgctgtatcttcaaatgggcagcctgagagctgaggacatggctgtgtattactgtgcgagatcattctatggttcggggacttattatgatacttttgatatgtggggccaagggacaatggtcaccgtctcttcagcctccaccaagggcccatcggtcttccccctggcgccctgctccaggagcacctccgagagcacagccgccctgggctgcctggtcaaggactacttccccgaaccggtgacggtgtcgtggaactcaggcgccctgaccagcggcgtgcacaccttcccggctgtcctacagtcctcaggactctactccctcagcagcgtggtgaccgtgccctccagcagcttgggcacgaagacctacacctgcaacgtagatcacaagcccagcaacaccaaggtggacaagagagttgagtccaaatatggtcccccatgcccaccctgcccagcacctgagttcctggggggaccatcagtcttcctgttccccccaaaacccaaggacactctcatgatctcccggacccctgaggtcacgtgcgtggtggtggacgtgagccaggaagaccccgaggtccagttcaactggtacgtggatggcgtggaggtgcataatgccaagacaaagccgcgggaggagcagttcaacagcacgtaccgtgtggtcagcgtcctcaccgtcctgcaccaggactggctgaacggcaaggagtacaagtgcaaggtctccaacaaaggcctcccgtcctccatcgagaaaaccatctccaaagccaaagggcagccccgagagccacaggtgtacaccctgcccccatcccaggaggagatgaccaagaaccaggtcagcctgacctgcctggtcaaaggcttctaccccagcgacatcgccgtggagtgggagagcaatgggcagccggagaacaactacaagaccacgcctcccgtgctggactccgacggctccttcttcctctacagcaggctcaccgtggacaagagcaggtggcaggaggggaatgtcttctcatgctccgtgatgcatgaggctctgcacaaccactacacacagaagtccctctccctgtctctgggtaaatga

SEQ ID NO: 115 - protein, 450 aa, Homo sapiens
EVQLVESGGGLVQPGGSLRLSCAASGFTFNNYAMHWVRQAPGKGLEYVSSISSSGGSTYYEDSVKGRFTISRDNSKNTLYLQMGSLRAEDMAVYYCARSFYGSGTYYDTFDMWGQGTMVTVSSASTKGPSVFPLAPCSRSTSESTAALGCLVKDYFPEPVTVSWNSGALTSGVHTFPAVLQSSGLYSLSSVVTVPSSSLGTKTYTCNVDHKPSNTKVDKRVESKYGPPCPPCPAPEFLGGPSVFLFPPKPKDTLMISRTPEVTCVVVDVSQEDPEVQFNWYVDGVEVHNAKTKPREEQFNSTYRVVSVLTVLHQDWLNGKEYKCKVSNKGLPSSIEKTISKAKGQPREPQVYTLPPSQEEMTKNQVSLTCLVKGFYPSDIAVEWESNGQPENNYKTTPPVLDSDGSFFLYSRLTVDKSRWQEGNVFSCSVMHEALHNHYTQKSLSLSLGK

SEQ ID NO: 116 - DNA, 645 bp, Homo sapiens
  source 1..645: mol_type = other DNA
gacatccagatgacccagtctccatcctccctgtctgcatctataggagacagagtcaccatcacttgccgggcaagtcagagcattagcaggtatttaaattggtatcagcagaaaccagggaaagcccctaagctcctgatctatgctgcatccagtttgcaaagtggggtcccatcaaggttcagtgccagtggatctgggacagatttcactctcaccatcagcagtctgcaacctgaagattttgcaacttactactgtcaacagagttacagtaccccgttcacttttggccaggggaccaagctggagatcaaacgaactgtggctgcaccatctgtcttcatcttcccgccatctgatgagcagttgaaatctggaactgcctctgttgtgtgcctgctgaataacttctatcccagagaggccaaagtacagtggaaggtggataacgccctccaatcgggtaactcccaggagagtgtcacagagcaggacagcaaggacagcacctacagcctcagcagcaccctgacgctgagcaaagcagactacgagaaacacaaagtctacgcctgcgaagtcacccatcagggcctgagctcgcccgtcacaaagagcttcaacaggggagagtgttag

SEQ ID NO: 117 - protein, 214 aa, Homo sapiens
DIQMTQSPSSLSASIGDRVTITCRASQSISRYLNWYQQKPGKAPKLLIYAASSLQSGVPSRFSASGSGTDFTLTISSLQPEDFATYYCQQSYSTPFTFGQGTKLEIKRTVAAPSVFIFPPSDEQLKSGTASVVCLLNNFYPREAKVQWKVDNALQSGNSQESVTEQDSKDSTYSLSSTLTLSKADYEKHKVYACEVTHQGLSSPVTKSFNRGEC

SEQ ID NO: 118 - DNA, 342 bp, Homo sapiens
  source 1..342: mol_type = other DNA
caggtgcagctggtggagtctgggggagacttggtcaagcctggggggtccctgagactctcctgtgcaacctctggattcaccttcagtgacttttacatgacctggatccgccaggctccagggaagggattggagtggatttcatatataagtaatagtgggagtatcgtgaagtacgcagactctgtgaagggccgattcaccatttccagggataacgccaagaactcactgtatctgcaaatgaacagcctgagagccgaggacacggccatttattactgtgcgcggttttatggtgacagatggggccagggaaccctggtcaccgtctcctca

SEQ ID NO: 119 - protein, 114 aa, Homo sapiens
QVQLVESGGDLVKPGGSLRLSCATSGFTFSDFYMTWIRQAPGKGLEWISYISNSGSIVKYADSVKGRFTISRDNAKNSLYLQMNSLRAEDTAIYYCARFYGDRWGQGTLVTVSS

SEQ ID NO: 120 - DNA, 24 bp, Homo sapiens
  source 1..24: mol_type = other DNA
ggattcaccttcagtgacttttac

SEQ ID NO: 121 - protein, 8 aa, Homo sapiens
GFTFSDFY

SEQ ID NO: 122 - DNA, 24 bp, Homo sapiens
  source 1..24: mol_type = other DNA
ataagtaatagtgggagtatcgtg

SEQ ID NO: 123 - protein, 8 aa, Homo sapiens
ISNSGSIV

SEQ ID NO: 124 - DNA, 21 bp, Homo sapiens
  source 1..21: mol_type = other DNA
gcgcggttttatggtgacaga

SEQ ID NO: 125 - protein, 7 aa, Homo sapiens
ARFYGDR

SEQ ID NO: 126 - DNA, 321 bp, Homo sapiens
  source 1..321: mol_type = other DNA
gacatccagttgacccagtctccatctttcctgtctgcatctgtaggagacagagtcaccatcacttgctgggccagtcagggcattagcacttttttagcctggtatcagcaaaagccgggtaaagcccctaagctcctgatctatgctgcatctactttacaaagtggggtcccatcgcgattcagcggcagcggatctgggacagatttcactctcacaatcagcagcctgcagcctgaagattttgcaacttatcactgtcaacaacttaataattacccgtggacgttcggccaagggaccaaggtggaaatcaaa

SEQ ID NO: 127 - protein, 107 aa, Homo sapiens
DIQLTQSPSFLSASVGDRVTITCWASQGISTFLAWYQQKPGKAPKLLIYAASTLQSGVPSRFSGSGSGTDFTLTISSLQPEDFATYHCQQLNNYPWTFGQGTKVEIK

SEQ ID NO: 128 - DNA, 18 bp, Homo sapiens
  source 1..18: mol_type = other DNA
cagggcattagcactttt

SEQ ID NO: 129 - protein, 6 aa, Homo sapiens
QGISTF

SEQ ID NO: 130 - skipped

SEQ ID NO: 131 - DNA, 27 bp, Homo sapiens
  source 1..27: mol_type = other DNA
caacaacttaataattacccgtggacg

SEQ ID NO: 132 - protein, 9 aa, Homo sapiens
QQLNNYPWT

SEQ ID NO: 133 - DNA, 1326 bp, Homo sapiens
  source 1..1326: mol_type = other DNA
caggtgcagctggtggagtctgggggagacttggtcaagcctggggggtccctgagactctcctgtgcaacctctggattcaccttcagtgacttttacatgacctggatccgccaggctccagggaagggattggagtggatttcatatataagtaatagtgggagtatcgtgaagtacgcagactctgtgaagggccgattcaccatttccagggataacgccaagaactcactgtatctgcaaatgaacagcctgagagccgaggacacggccatttattactgtgcgcggttttatggtgacagatggggccagggaaccctggtcaccgtctcctcagcctccaccaagggcccatcggtcttccccctggcgccctgctccaggagcacctccgagagcacagccgccctgggctgcctggtcaaggactacttccccgaaccggtgacggtgtcgtggaactcaggcgccctgaccagcggcgtgcacaccttcccggctgtcctacagtcctcaggactctactccctcagcagcgtggtgaccgtgccctccagcagcttgggcacgaagacctacacctgcaacgtagatcacaagcccagcaacaccaaggtggacaagagagttgagtccaaatatggtcccccatgcccaccctgcccagcacctgagttcctggggggaccatcagtcttcctgttccccccaaaacccaaggacactctcatgatctcccggacccctgaggtcacgtgcgtggtggtggacgtgagccaggaagaccccgaggtccagttcaactggtacgtggatggcgtggaggtgcataatgccaagacaaagccgcgggaggagcagttcaacagcacgtaccgtgtggtcagcgtcctcaccgtcctgcaccaggactggctgaacggcaaggagtacaagtgcaaggtctccaacaaaggcctcccgtcctccatcgagaaaaccatctccaaagccaaagggcagccccgagagccacaggtgtacaccctgcccccatcccaggaggagatgaccaagaaccaggtcagcctgacctgcctggtcaaaggcttctaccccagcgacatcgccgtggagtgggagagcaatgggcagccggagaacaactacaagaccacgcctcccgtgctggactccgacggctccttcttcctctacagcaggctcaccgtggacaagagcaggtggcaggaggggaatgtcttctcatgctccgtgatgcatgaggctctgcacaaccactacacacagaagtccctctccctgtctctgggtaaatga

SEQ ID NO: 134 - protein, 441 aa, Homo sapiens
QVQLVESGGDLVKPGGSLRLSCATSGFTFSDFYMTWIRQAPGKGLEWISYISNSGSIVKYADSVKGRFTISRDNAKNSLYLQMNSLRAEDTAIYYCARFYGDRWGQGTLVTVSSASTKGPSVFPLAPCSRSTSESTAALGCLVKDYFPEPVTVSWNSGALTSGVHTFPAVLQSSGLYSLSSVVTVPSSSLGTKTYTCNVDHKPSNTKVDKRVESKYGPPCPPCPAPEFLGGPSVFLFPPKPKDTLMISRTPEVTCVVVDVSQEDPEVQFNWYVDGVEVHNAKTKPREEQFNSTYRVVSVLTVLHQDWLNGKEYKCKVSNKGLPSSIEKTISKAKGQPREPQVYTLPPSQEEMTKNQVSLTCLVKGFYPSDIAVEWESNGQPENNYKTTPPVLDSDGSFFLYSRLTVDKSRWQEGNVFSCSVMHEALHNHYTQKSLSLSLGK

SEQ ID NO: 135 - DNA, 645 bp, Homo sapiens
  source 1..645: mol_type = other DNA
gacatccagttgacccagtctccatctttcctgtctgcatctgtaggagacagagtcaccatcacttgctgggccagtcagggcattagcacttttttagcctggtatcagcaaaagccgggtaaagcccctaagctcctgatctatgctgcatctactttacaaagtggggtcccatcgcgattcagcggcagcggatctgggacagatttcactctcacaatcagcagcctgcagcctgaagattttgcaacttatcactgtcaacaacttaataattacccgtggacgttcggccaagggaccaaggtggaaatcaaacgaactgtggctgcaccatctgtcttcatcttcccgccatctgatgagcagttgaaatctggaactgcctctgttgtgtgcctgctgaataacttctatcccagagaggccaaagtacagtggaaggtggataacgccctccaatcgggtaactcccaggagagtgtcacagagcaggacagcaaggacagcacctacagcctcagcagcaccctgacgctgagcaaagcagactacgagaaacacaaagtctacgcctgcgaagtcacccatcagggcctgagctcgcccgtcacaaagagcttcaacaggggagagtgttag

SEQ ID NO: 136 - protein, 214 aa, Homo sapiens
DIQLTQSPSFLSASVGDRVTITCWASQGISTFLAWYQQKPGKAPKLLIYAASTLQSGVPSRFSGSGSGTDFTLTISSLQPEDFATYHCQQLNNYPWTFGQGTKVEIKRTVAAPSVFIFPPSDEQLKSGTASVVCLLNNFYPREAKVQWKVDNALQSGNSQESVTEQDSKDSTYSLSSTLTLSKADYEKHKVYACEVTHQGLSSPVTKSFNRGEC

SEQ ID NO: 137 - DNA, 342 bp, Homo sapiens
  source 1..342: mol_type = other DNA
caggtgcagctggtggagtctgggggaggcttggtcaagcctggagggtccctgagactctcctgtgaagcctctggattcaccttcaatgacttctatatgacctggatccgccaggctccagggaaggggctggagtggattgcatacatttctaagagtggtgataaaatgcgttatgcagactctgtgaagggccgattcagcacctccagggacaacgccaagaattcactatccttgcaaatgaatagcctgagagccgaggacacggccgtgtattattgtgcgagattctacggtgatatatggggccagggaaccctggtcaccgtctcctca

SEQ ID NO: 138 - protein, 114 aa, Homo sapiens
QVQLVESGGGLVKPGGSLRLSCEASGFTFNDFYMTWIRQAPGKGLEWIAYISKSGDKMRYADSVKGRFSTSRDNAKNSLSLQMNSLRAEDTAVYYCARFYGDIWGQGTLVTVSS

SEQ ID NO: 139 - DNA, 24 bp, Homo sapiens
  source 1..24: mol_type = other DNA
ggattcaccttcaatgacttctat

SEQ ID NO: 140 - protein, 8 aa, Homo sapiens
GFTFNDFY

SEQ ID NO: 141 - DNA, 24 bp, Homo sapiens
  source 1..24: mol_type = other DNA
atttctaagagtggtgataaaatg

SEQ ID NO: 142 - protein, 8 aa, Homo sapiens
ISKSGDKM

SEQ ID NO: 143 - DNA, 21 bp, Homo sapiens
  source 1..21: mol_type = other DNA
gcgagattctacggtgatata

SEQ ID NO: 144 - protein, 7 aa, Homo sapiens
ARFYGDI

SEQ ID NO: 145 - DNA, 321 bp, Homo sapiens
  source 1..321: mol_type = other DNA
gacatccagttgacccagtctccatccttcctgtctgcatctgtaggagacagagtcaccatcacttgctgggccagtcaggacattagcagttttttagtctggtatcagcaaaaaccagggaaagcccctaacctcctgatctatgctgcatccgctttgcagagtggggtcccatcaaggttcagcggcagtggatctgggacagaattcactctcacaatcagcagcctgcagcctgaagattttgcaagttattactgtgaacagcttaataattatccgtggacgttcggccaagggaccaaggtggaaatcaaa

SEQ ID NO: 146 - protein, 107 aa, Homo sapiens
DIQLTQSPSFLSASVGDRVTITCWASQDISSFLVWYQQKPGKAPNLLIYAASALQSGVPSRFSGSGSGTEFTLTISSLQPEDFASYYCEQLNNYPWTFGQGTKVEIK

SEQ ID NO: 147 - DNA, 18 bp, Homo sapiens
  source 1..18: mol_type = other DNA
caggacattagcagtttt

SEQ ID NO: 148 - protein, 6 aa, Homo sapiens
QDISSF

SEQ ID NO: 149 - DNA, 27 bp, Homo sapiens
  source 1..27: mol_type = other DNA
gaacagcttaataattatccgtggacg

SEQ ID NO: 150 - protein, 9 aa, Homo sapiens
EQLNNYPWT

SEQ ID NO: 151 - DNA, 1326 bp, Homo sapiens
  source 1..1326: mol_type = other DNA
caggtgcagctggtggagtctgggggaggcttggtcaagcctggagggtccctgagactctcctgtgaagcctctggattcaccttcaatgacttctatatgacctggatccgccaggctccagggaaggggctggagtggattgcatacatttctaagagtggtgataaaatgcgttatgcagactctgtgaagggccgattcagcacctccagggacaacgccaagaattcactatccttgcaaatgaatagcctgagagccgaggacacggccgtgtattattgtgcgagattctacggtgatatatggggccagggaaccctggtcaccgtctcctcagcctccaccaagggcccatcggtcttccccctggcgccctgctccaggagcacctccgagagcacagccgccctgggctgcctggtcaaggactacttccccgaaccggtgacggtgtcgtggaactcaggcgccctgaccagcggcgtgcacaccttcccggctgtcctacagtcctcaggactctactccctcagcagcgtggtgaccgtgccctccagcagcttgggcacgaagacctacacctgcaacgtagatcacaagcccagcaacaccaaggtggacaagagagttgagtccaaatatggtcccccatgcccaccctgcccagcacctgagttcctggggggaccatcagtcttcctgttccccccaaaacccaaggacactctcatgatctcccggacccctgaggtcacgtgcgtggtggtggacgtgagccaggaagaccccgaggtccagttcaactggtacgtggatggcgtggaggtgcataatgccaagacaaagccgcgggaggagcagttcaacagcacgtaccgtgtggtcagcgtcctcaccgtcctgcaccaggactggctgaacggcaaggagtacaagtgcaaggtctccaacaaaggcctcccgtcctccatcgagaaaaccatctccaaagccaaagggcagccccgagagccacaggtgtacaccctgcccccatcccaggaggagatgaccaagaaccaggtcagcctgacctgcctggtcaaaggcttctaccccagcgacatcgccgtggagtgggagagcaatgggcagccggagaacaactacaagaccacgcctcccgtgctggactccgacggctccttcttcctctacagcaggctcaccgtggacaagagcaggtggcaggaggggaatgtcttctcatgctccgtgatgcatgaggctctgcacaaccactacacacagaagtccctctccctgtctctgggtaaatga

SEQ ID NO: 152 - protein, 441 aa, Homo sapiens
QVQLVESGGGLVKPGGSLRLSCEASGFTFNDFYMTWIRQAPGKGLEWIAYISKSGDKMRYADSVKGRFSTSRDNAKNSLSLQMNSLRAEDTAVYYCARFYGDIWGQGTLVTVSSASTKGPSVFPLAPCSRSTSESTAALGCLVKDYFPEPVTVSWNSGALTSGVHTFPAVLQSSGLYSLSSVVTVPSSSLGTKTYTCNVDHKPSNTKVDKRVESKYGPPCPPCPAPEFLGGPSVFLFPPKPKDTLMISRTPEVTCVVVDVSQEDPEVQFNWYVDGVEVHNAKTKPREEQFNSTYRVVSVLTVLHQDWLNGKEYKCKVSNKGLPSSIEKTISKAKGQPREPQVYTLPPSQEEMTKNQVSLTCLVKGFYPSDIAVEWESNGQPENNYKTTPPVLDSDGSFFLYSRLTVDKSRWQEGNVFSCSVMHEALHNHYTQKSLSLSLGK

SEQ ID NO: 153 - DNA, 645 bp, Homo sapiens
  source 1..645: mol_type = other DNA
gacatccagttgacccagtctccatccttcctgtctgcatctgtaggagacagagtcaccatcacttgctgggccagtcaggacattagcagttttttagtctggtatcagcaaaaaccagggaaagcccctaacctcctgatctatgctgcatccgctttgcagagtggggtcccatcaaggttcagcggcagtggatctgggacagaattcactctcacaatcagcagcctgcagcctgaagattttgcaagttattactgtgaacagcttaataattatccgtggacgttcggccaagggaccaaggtggaaatcaaacgaactgtggctgcaccatctgtcttcatcttcccgccatctgatgagcagttgaaatctggaactgcctctgttgtgtgcctgctgaataacttctatcccagagaggccaaagtacagtggaaggtggataacgccctccaatcgggtaactcccaggagagtgtcacagagcaggacagcaaggacagcacctacagcctcagcagcaccctgacgctgagcaaagcagactacgagaaacacaaagtctacgcctgcgaagtcacccatcagggcctgagctcgcccgtcacaaagagcttcaacaggggagagtgttag

SEQ ID NO: 154 - protein, 214 aa, Homo sapiens
DIQLTQSPSFLSASVGDRVTITCWASQDISSFLVWYQQKPGKAPNLLIYAASALQSGVPSRFSGSGSGTEFTLTISSLQPEDFASYYCEQLNNYPWTFGQGTKVEIKRTVAAPSVFIFPPSDEQLKSGTASVVCLLNNFYPREAKVQWKVDNALQSGNSQESVTEQDSKDSTYSLSSTLTLSKADYEKHKVYACEVTHQGLSSPVTKSFNRGEC

SEQ ID NO: 155 - DNA, 375 bp, Homo sapiens
  source 1..375: mol_type = other DNA
gaggtgcagctggtggagtccgggggacgcttggtacagcctggggggtccctgagactctcctgtgaagcctctggattcacgtttagtaattatggcatgacctgggtccgccaggctccagggaaggggctggaatgggtctcagttattagtggcagtgataatagaaaatactatgcagagtccgtgaagggccggttcaccatctccagagacaattccaaaaacacactatatctgcaaatgaatagcctgagagccgaggacacggccgtctattactgtgcaaaattgggatatagtcgttcgtccaaggacttctactacggaatggacgtctggggccaagggaccacggtcaccgtctcctca

SEQ ID NO: 156 - protein, 125 aa, Homo sapiens
EVQLVESGGRLVQPGGSLRLSCEASGFTFSNYGMTWVRQAPGKGLEWVSVISGSDNRKYYAESVKGRFTISRDNSKNTLYLQMNSLRAEDTAVYYCAKLGYSRSSKDFYYGMDVWGQGTTVTVSS

SEQ ID NO: 157 - DNA, 24 bp, Homo sapiens
  source 1..24: mol_type = other DNA
ggattcacgtttagtaattatggc

SEQ ID NO: 158 - protein, 8 aa, Homo sapiens
GFTFSNYG

SEQ ID NO: 159 - DNA, 24 bp, Homo sapiens
  source 1..24: mol_type = other DNA
attagtggcagtgataatagaaaa

SEQ ID NO: 160 - protein, 8 aa, Homo sapiens
ISGSDNRK

SEQ ID NO: 161 - DNA, 54 bp, Homo sapiens
  source 1..54: mol_type = other DNA
gcaaaattgggatatagtcgttcgtccaaggacttctactacggaatggacgtc

SEQ ID NO: 162 - protein, 18 aa, Homo sapiens
AKLGYSRSSKDFYYGMDV

SEQ ID NO: 163 - DNA, 339 bp, Homo sapiens
  source 1..339: mol_type = other DNA
gacatcgtgatgacccagtctccagactccctggctgtgtctctgggcgagagggccaccatcaactgcaagtccagccagagtgttttatacaattccaataataggaactacttagtttggtaccagcagaaaccaggacagtctcctaagttgctcatttactgggcatctacccgggaatccggggtccctgaccggttcagtggcagcgggtctgggacagatttcactctcaccatcagcagcctgcaggctgaagatgtggcagtgtattactgtcagcaatattataatgttccgtacacttttggccaggggaccaagctggagatcaaa

SEQ ID NO: 164 - protein, 113 aa, Homo sapiens
DIVMTQSPDSLAVSLGERATINCKSSQSVLYNSNNRNYLVWYQQKPGQSPKLLIYWASTRESGVPDRFSGSGSGTDFTLTISSLQAEDVAVYYCQQYYNVPYTFGQGTKLEIK

SEQ ID NO: 165 - DNA, 36 bp, Homo sapiens
  source 1..36: mol_type = other DNA
cagagtgttttatacaattccaataataggaactac

SEQ ID NO: 166 - protein, 12 aa, Homo sapiens
QSVLYNSNNRNY

SEQ ID NO: 167 - DNA, 27 bp, Homo sapiens
  source 1..27: mol_type = other DNA
cagcaatattataatgttccgtacact

SEQ ID NO: 168 - protein, 9 aa, Homo sapiens
QQYYNVPYT

SEQ ID NO: 169 - DNA, 1359 bp, Homo sapiens
  source 1..1359: mol_type = other DNA
gaggtgcagctggtggagtccgggggacgcttggtacagcctggggggtccctgagactctcctgtgaagcctctggattcacgtttagtaattatggcatgacctgggtccgccaggctccagggaaggggctggaatgggtctcagttattagtggcagtgataatagaaaatactatgcagagtccgtgaagggccggttcaccatctccagagacaattccaaaaacacactatatctgcaaatgaatagcctgagagccgaggacacggccgtctattactgtgcaaaattgggatatagtcgttcgtccaaggacttctactacggaatggacgtctggggccaagggaccacggtcaccgtctcctcagcctccaccaagggcccatcggtcttccccctggcgccctgctccaggagcacctccgagagcacagccgccctgggctgcctggtcaaggactacttccccgaaccggtgacggtgtcgtggaactcaggcgccctgaccagcggcgtgcacaccttcccggctgtcctacagtcctcaggactctactccctcagcagcgtggtgaccgtgccctccagcagcttgggcacgaagacctacacctgcaacgtagatcacaagcccagcaacaccaaggtggacaagagagttgagtccaaatatggtcccccatgcccaccctgcccagcacctgagttcctggggggaccatcagtcttcctgttccccccaaaacccaaggacactctcatgatctcccggacccctgaggtcacgtgcgtggtggtggacgtgagccaggaagaccccgaggtccagttcaactggtacgtggatggcgtggaggtgcataatgccaagacaaagccgcgggaggagcagttcaacagcacgtaccgtgtggtcagcgtcctcaccgtcctgcaccaggactggctgaacggcaaggagtacaagtgcaaggtctccaacaaaggcctcccgtcctccatcgagaaaaccatctccaaagccaaagggcagccccgagagccacaggtgtacaccctgcccccatcccaggaggagatgaccaagaaccaggtcagcctgacctgcctggtcaaaggcttctaccccagcgacatcgccgtggagtgggagagcaatgggcagccggagaacaactacaagaccacgcctcccgtgctggactccgacggctccttcttcctctacagcaggctcaccgtggacaagagcaggtggcaggaggggaatgtcttctcatgctccgtgatgcatgaggctctgcacaaccactacacacagaagtccctctccctgtctctgggtaaatga

SEQ ID NO: 170 - protein, 452 aa, Homo sapiens
EVQLVESGGRLVQPGGSLRLSCEASGFTFSNYGMTWVRQAPGKGLEWVSVISGSDNRKYYAESVKGRFTISRDNSKNTLYLQMNSLRAEDTAVYYCAKLGYSRSSKDFYYGMDVWGQGTTVTVSSASTKGPSVFPLAPCSRSTSESTAALGCLVKDYFPEPVTVSWNSGALTSGVHTFPAVLQSSGLYSLSSVVTVPSSSLGTKTYTCNVDHKPSNTKVDKRVESKYGPPCPPCPAPEFLGGPSVFLFPPKPKDTLMISRTPEVTCVVVDVSQEDPEVQFNWYVDGVEVHNAKTKPREEQFNSTYRVVSVLTVLHQDWLNGKEYKCKVSNKGLPSSIEKTISKAKGQPREPQVYTLPPSQEEMTKNQVSLTCLVKGFYPSDIAVEWESNGQPENNYKTTPPVLDSDGSFFLYSRLTVDKSRWQEGNVFSCSVMHEALHNHYTQKSLSLSLGK

SEQ ID NO: 171 - DNA, 663 bp, Homo sapiens
  source 1..663: mol_type = other DNA
gacatcgtgatgacccagtctccagactccctggctgtgtctctgggcgagagggccaccatcaactgcaagtccagccagagtgttttatacaattccaataataggaactacttagtttggtaccagcagaaaccaggacagtctcctaagttgctcatttactgggcatctacccgggaatccggggtccctgaccggttcagtggcagcgggtctgggacagatttcactctcaccatcagcagcctgcaggctgaagatgtggcagtgtattactgtcagcaatattataatgttccgtacacttttggccaggggaccaagctggagatcaaacgaactgtggctgcaccatctgtcttcatcttcccgccatctgatgagcagttgaaatctggaactgcctctgttgtgtgcctgctgaataacttctatcccagagaggccaaagtacagtggaaggtggataacgccctccaatcgggtaactcccaggagagtgtcacagagcaggacagcaaggacagcacctacagcctcagcagcaccctgacgctgagcaaagcagactacgagaaacacaaagtctacgcctgcgaagtcacccatcagggcctgagctcgcccgtcacaaagagcttcaacaggggagagtgttag

SEQ ID NO: 172 - protein, 220 aa, Homo sapiens
DIVMTQSPDSLAVSLGERATINCKSSQSVLYNSNNRNYLVWYQQKPGQSPKLLIYWASTRESGVPDRFSGSGSGTDFTLTISSLQAEDVAVYYCQQYYNVPYTFGQGTKLEIKRTVAAPSVFIFPPSDEQLKSGTASVVCLLNNFYPREAKVQWKVDNALQSGNSQESVTEQDSKDSTYSLSSTLTLSKADYEKHKVYACEVTHQGLSSPVTKSFNRGEC

SEQ ID NO: 173 - DNA, 348 bp, Homo sapiens
  source 1..348: mol_type = other DNA
gaggtgcagctggtggagtctgggggaggtgtggtacggcctggggggtccctgagactctcctgtgcagcctctggattcacctttgatgattatggcatgagctgggtccgccaagctccagggaaggggctggagtggatctcttctattaataggaatggtggtagcgcagattatgcagactctgtgaagggccgattcaccatctccagagacaacgccaagaactccctctttctgcaaatgagcagtctgagagccgaggacacggccctctatcactgtgcgagcggggagtttcgctttgactactggggccagggaaccctggtcaccgtctcctca

SEQ ID NO: 174 - protein, 116 aa, Homo sapiens
EVQLVESGGGVVRPGGSLRLSCAASGFTFDDYGMSWVRQAPGKGLEWISSINRNGGSADYADSVKGRFTISRDNAKNSLFLQMSSLRAEDTALYHCASGEFRFDYWGQGTLVTVSS

SEQ ID NO: 175 - DNA, 24 bp, Homo sapiens
  source 1..24: mol_type = other DNA
ggattcacctttgatgattatggc

SEQ ID NO: 176 - protein, 8 aa, Homo sapiens
GFTFDDYG

SEQ ID NO: 177 - DNA, 24 bp, Homo sapiens
  source 1..24: mol_type = other DNA
attaataggaatggtggtagcgca

SEQ ID NO: 178 - protein, 8 aa, Homo sapiens
INRNGGSA

SEQ ID NO: 179 - DNA, 27 bp, Homo sapiens
  source 1..27: mol_type = other DNA
gcgagcggggagtttcgctttgactac

SEQ ID NO: 180 - protein, 9 aa, Homo sapiens
ASGEFRFDY

SEQ ID NO: 181 - DNA, 324 bp, Homo sapiens
  source 1..324: mol_type = other DNA
gacatccagatgacccagtctccatcctccctgtctgcatctgtaggagacagagtcaccatcacttgccgggcaagtcagagcattagcagctatttaaattggtatcagcagaaaccagggaaagcccctaagctcctgatctatgctgcatccagtttgcaaagtggggtcccgtcaaggttcagtggcagtggatctgggacagatttcactctcaccatcagcagtctgcaacctgaagattttgcaacttactactgtcaacagagttacagtacccctccgatcaccttcggccaagggacacgactggagattaaa

SEQ ID NO: 182 - protein, 108 aa, Homo sapiens
DIQMTQSPSSLSASVGDRVTITCRASQSISSYLNWYQQKPGKAPKLLIYAASSLQSGVPSRFSGSGSGTDFTLTISSLQPEDFATYYCQQSYSTPPITFGQGTRLEIK

SEQ ID NO: 183 - DNA, 30 bp, Homo sapiens
  source 1..30: mol_type = other DNA
caacagagttacagtacccctccgatcacc

SEQ ID NO: 184 - protein, 10 aa, Homo sapiens
QQSYSTPPIT

SEQ ID NO: 185 - DNA, 1332 bp, Homo sapiens
  source 1..1332: mol_type = other DNA
gaggtgcagctggtggagtctgggggaggtgtggtacggcctggggggtccctgagactctcctgtgcagcctctggattcacctttgatgattatggcatgagctgggtccgccaagctccagggaaggggctggagtggatctcttctattaataggaatggtggtagcgcagattatgcagactctgtgaagggccgattcaccatctccagagacaacgccaagaactccctctttctgcaaatgagcagtctgagagccgaggacacggccctctatcactgtgcgagcggggagtttcgctttgactactggggccagggaaccctggtcaccgtctcctcagcctccaccaagggcccatcggtcttccccctggcgccctgctccaggagcacctccgagagcacagccgccctgggctgcctggtcaaggactacttccccgaaccggtgacggtgtcgtggaactcaggcgccctgaccagcggcgtgcacaccttcccggctgtcctacagtcctcaggactctactccctcagcagcgtggtgaccgtgccctccagcagcttgggcacgaagacctacacctgcaacgtagatcacaagcccagcaacaccaaggtggacaagagagttgagtccaaatatggtcccccatgcccaccctgcccagcacctgagttcctggggggaccatcagtcttcctgttccccccaaaacccaaggacactctcatgatctcccggacccctgaggtcacgtgcgtggtggtggacgtgagccaggaagaccccgaggtccagttcaactggtacgtggatggcgtggaggtgcataatgccaagacaaagccgcgggaggagcagttcaacagcacgtaccgtgtggtcagcgtcctcaccgtcctgcaccaggactggctgaacggcaaggagtacaagtgcaaggtctccaacaaaggcctcccgtcctccatcgagaaaaccatctccaaagccaaagggcagccccgagagccacaggtgtacaccctgcccccatcccaggaggagatgaccaagaaccaggtcagcctgacctgcctggtcaaaggcttctaccccagcgacatcgccgtggagtgggagagcaatgggcagccggagaacaactacaagaccacgcctcccgtgctggactccgacggctccttcttcctctacagcaggctcaccgtggacaagagcaggtggcaggaggggaatgtcttctcatgctccgtgatgcatgaggctctgcacaaccactacacacagaagtccctctccctgtctctgggtaaatga

SEQ ID NO: 186 - protein, 443 aa, Homo sapiens
EVQLVESGGGVVRPGGSLRLSCAASGFTFDDYGMSWVRQAPGKGLEWISSINRNGGSADYADSVKGRFTISRDNAKNSLFLQMSSLRAEDTALYHCASGEFRFDYWGQGTLVTVSSASTKGPSVFPLAPCSRSTSESTAALGCLVKDYFPEPVTVSWNSGALTSGVHTFPAVLQSSGLYSLSSVVTVPSSSLGTKTYTCNVDHKPSNTKVDKRVESKYGPPCPPCPAPEFLGGPSVFLFPPKPKDTLMISRTPEVTCVVVDVSQEDPEVQFNWYVDGVEVHNAKTKPREEQFNSTYRVVSVLTVLHQDWLNGKEYKCKVSNKGLPSSIEKTISKAKGQPREPQVYTLPPSQEEMTKNQVSLTCLVKGFYPSDIAVEWESNGQPENNYKTTPPVLDSDGSFFLYSRLTVDKSRWQEGNVFSCSVMHEALHNHYTQKSLSLSLGK

SEQ ID NO: 187 - DNA, 648 bp, Homo sapiens
  source 1..648: mol_type = other DNA
gacatccagatgacccagtctccatcctccctgtctgcatctgtaggagacagagtcaccatcacttgccgggcaagtcagagcattagcagctatttaaattggtatcagcagaaaccagggaaagcccctaagctcctgatctatgctgcatccagtttgcaaagtggggtcccgtcaaggttcagtggcagtggatctgggacagatttcactctcaccatcagcagtctgcaacctgaagattttgcaacttactactgtcaacagagttacagtacccctccgatcaccttcggccaagggacacgactggagattaaacgaactgtggctgcaccatctgtcttcatcttcccgccatctgatgagcagttgaaatctggaactgcctctgttgtgtgcctgctgaataacttctatcccagagaggccaaagtacagtggaaggtggataacgccctccaatcgggtaactcccaggagagtgtcacagagcaggacagcaaggacagcacctacagcctcagcagcaccctgacgctgagcaaagcagactacgagaaacacaaagtctacgcctgcgaagtcacccatcagggcctgagctcgcccgtcacaaagagcttcaacaggggagagtgttag

SEQ ID NO: 188 - protein, 215 aa, Homo sapiens
DIQMTQSPSSLSASVGDRVTITCRASQSISSYLNWYQQKPGKAPKLLIYAASSLQSGVPSRFSGSGSGTDFTLTISSLQPEDFATYYCQQSYSTPPITFGQGTRLEIKRTVAAPSVFIFPPSDEQLKSGTASVVCLLNNFYPREAKVQWKVDNALQSGNSQESVTEQDSKDSTYSLSSTLTLSKADYEKHKVYACEVTHQGLSSPVTKSFNRGEC

SEQ ID NO: 189 - DNA, 348 bp, Homo sapiens
  source 1..348: mol_type = other DNA
gaagtgcagctggtggagtctgggggaggcttggtacagcctggcaggtccctgagactctcctgtgcagcctctggattcacccttgaagattatgccatgcactgggtccggcaagctccagggaagggcctggaatgggtctcaggtattagttggaatagaggtagcacaggctatgcggactctgtgaagggccgattcaccatctcaagagacaacgccaagaactccctgtatctgcaaatgaccagtctgagagctgaggacacggccttgtattactgtgcaaaaggattctacagtatggacgtctggggccaagggaccacggtcaccgtctcctca

SEQ ID NO: 190 - protein, 116 aa, Homo sapiens
EVQLVESGGGLVQPGRSLRLSCAASGFTLEDYAMHWVRQAPGKGLEWVSGISWNRGSTGYADSVKGRFTISRDNAKNSLYLQMTSLRAEDTALYYCAKGFYSMDVWGQGTTVTVSS

SEQ ID NO: 191 - DNA, 24 bp, Homo sapiens
  source 1..24: mol_type = other DNA
ggattcacccttgaagattatgcc

SEQ ID NO: 192 - protein, 8 aa, Homo sapiens
GFTLEDYA

SEQ ID NO: 193 - DNA, 24 bp, Homo sapiens
  source 1..24: mol_type = other DNA
attagttggaatagaggtagcaca

SEQ ID NO: 194 - protein, 8 aa, Homo sapiens
ISWNRGST

SEQ ID NO: 195 - DNA, 27 bp, Homo sapiens
  source 1..27: mol_type = other DNA
gcaaaaggattctacagtatggacgtc

SEQ ID NO: 196 - protein, 9 aa, Homo sapiens
AKGFYSMDV

SEQ ID NO: 197 - DNA, 1332 bp, Homo sapiens
  source 1..1332: mol_type = other DNA
gaagtgcagctggtggagtctgggggaggcttggtacagcctggcaggtccctgagactctcctgtgcagcctctggattcacccttgaagattatgccatgcactgggtccggcaagctccagggaagggcctggaatgggtctcaggtattagttggaatagaggtagcacaggctatgcggactctgtgaagggccgattcaccatctcaagagacaacgccaagaactccctgtatctgcaaatgaccagtctgagagctgaggacacggccttgtattactgtgcaaaaggattctacagtatggacgtctggggccaagggaccacggtcaccgtctcctcagcctccaccaagggcccatcggtcttccccctggcgccctgctccaggagcacctccgagagcacagccgccctgggctgcctggtcaaggactacttccccgaaccggtgacggtgtcgtggaactcaggcgccctgaccagcggcgtgcacaccttcccggctgtcctacagtcctcaggactctactccctcagcagcgtggtgaccgtgccctccagcagcttgggcacgaagacctacacctgcaacgtagatcacaagcccagcaacaccaaggtggacaagagagttgagtccaaatatggtcccccatgcccaccctgcccagcacctgagttcctggggggaccatcagtcttcctgttccccccaaaacccaaggacactctcatgatctcccggacccctgaggtcacgtgcgtggtggtggacgtgagccaggaagaccccgaggtccagttcaactggtacgtggatggcgtggaggtgcataatgccaagacaaagccgcgggaggagcagttcaacagcacgtaccgtgtggtcagcgtcctcaccgtcctgcaccaggactggctgaacggcaaggagtacaagtgcaaggtctccaacaaaggcctcccgtcctccatcgagaaaaccatctccaaagccaaagggcagccccgagagccacaggtgtacaccctgcccccatcccaggaggagatgaccaagaaccaggtcagcctgacctgcctggtcaaaggcttctaccccagcgacatcgccgtggagtgggagagcaatgggcagccggagaacaactacaagaccacgcctcccgtgctggactccgacggctccttcttcctctacagcaggctcaccgtggacaagagcaggtggcaggaggggaatgtcttctcatgctccgtgatgcatgaggctctgcacaaccactacacacagaagtccctctccctgtctctgggtaaatga

SEQ ID NO: 198 - protein, 443 aa, Homo sapiens
EVQLVESGGGLVQPGRSLRLSCAASGFTLEDYAMHWVRQAPGKGLEWVSGISWNRGSTGYADSVKGRFTISRDNAKNSLYLQMTSLRAEDTALYYCAKGFYSMDVWGQGTTVTVSSASTKGPSVFPLAPCSRSTSESTAALGCLVKDYFPEPVTVSWNSGALTSGVHTFPAVLQSSGLYSLSSVVTVPSSSLGTKTYTCNVDHKPSNTKVDKRVESKYGPPCPPCPAPEFLGGPSVFLFPPKPKDTLMISRTPEVTCVVVDVSQEDPEVQFNWYVDGVEVHNAKTKPREEQFNSTYRVVSVLTVLHQDWLNGKEYKCKVSNKGLPSSIEKTISKAKGQPREPQVYTLPPSQEEMTKNQVSLTCLVKGFYPSDIAVEWESNGQPENNYKTTPPVLDSDGSFFLYSRLTVDKSRWQEGNVFSCSVMHEALHNHYTQKSLSLSLGK

SEQ ID NO: 199 - DNA, 363 bp, Homo sapiens
  source 1..363: mol_type = other DNA
caggtacagctgcagcagtcaggtccaggactggtgaagccctcgcagaccctctcactcacctgtgccatctccggtgacagtgtctctagcaacattgctgcttggaactggatcaggctgtccccatcgagaggccttgagtggctgggaaggacattcttcaggtccacgtggttttatgattattcactatctgtgaaaggtcgcataaccatcaacccagacacatccaagaaccagttctccctgcacctgaactctgtgactcccgaggacgcggctgtgtattattgtgcaagaacggggcgacggtggtctcttgactactggggccagggaaccctggtcaccgtctcctca

SEQ ID NO: 200 - protein, 121 aa, Homo sapiens
QVQLQQSGPGLVKPSQTLSLTCAISGDSVSSNIAAWNWIRLSPSRGLEWLGRTFFRSTWFYDYSLSVKGRITINPDTSKNQFSLHLNSVTPEDAAVYYCARTGRRWSLDYWGQGTLVTVSS

SEQ ID NO: 201 - DNA, 30 bp, Homo sapiens
  source 1..30: mol_type = other DNA
ggtgacagtgtctctagcaacattgctgct

SEQ ID NO: 202 - protein, 10 aa, Homo sapiens
GDSVSSNIAA

SEQ ID NO: 203 - DNA, 27 bp, Homo sapiens
  source 1..27: mol_type = other DNA
acattcttcaggtccacgtggttttat

SEQ ID NO: 204 - protein, 9 aa, Homo sapiens
TFFRSTWFY

SEQ ID NO: 205 - DNA, 33 bp, Homo sapiens
  source 1..33: mol_type = other DNA
gcaagaacggggcgacggtggtctcttgactac

SEQ ID NO: 206 - protein, 11 aa, Homo sapiens
ARTGRRWSLDY

SEQ ID NO: 207 - DNA, 1347 bp, Homo sapiens
  source 1..1347: mol_type = other DNA
caggtacagctgcagcagtcaggtccaggactggtgaagccctcgcagaccctctcactcacctgtgccatctccggtgacagtgtctctagcaacattgctgcttggaactggatcaggctgtccccatcgagaggccttgagtggctgggaaggacattcttcaggtccacgtggttttatgattattcactatctgtgaaaggtcgcataaccatcaacccagacacatccaagaaccagttctccctgcacctgaactctgtgactcccgaggacgcggctgtgtattattgtgcaagaacggggcgacggtggtctcttgactactggggccagggaaccctggtcaccgtctcctcagcctccaccaagggcccatcggtcttccccctggcgccctgctccaggagcacctccgagagcacagccgccctgggctgcctggtcaaggactacttccccgaaccggtgacggtgtcgtggaactcaggcgccctgaccagcggcgtgcacaccttcccggctgtcctacagtcctcaggactctactccctcagcagcgtggtgaccgtgccctccagcagcttgggcacgaagacctacacctgcaacgtagatcacaagcccagcaacaccaaggtggacaagagagttgagtccaaatatggtcccccatgcccaccctgcccagcacctgagttcctggggggaccatcagtcttcctgttccccccaaaacccaaggacactctcatgatctcccggacccctgaggtcacgtgcgtggtggtggacgtgagccaggaagaccccgaggtccagttcaactggtacgtggatggcgtggaggtgcataatgccaagacaaagccgcgggaggagcagttcaacagcacgtaccgtgtggtcagcgtcctcaccgtcctgcaccaggactggctgaacggcaaggagtacaagtgcaaggtctccaacaaaggcctcccgtcctccatcgagaaaaccatctccaaagccaaagggcagccccgagagccacaggtgtacaccctgcccccatcccaggaggagatgaccaagaaccaggtcagcctgacctgcctggtcaaaggcttctaccccagcgacatcgccgtggagtgggagagcaatgggcagccggagaacaactacaagaccacgcctcccgtgctggactccgacggctccttcttcctctacagcaggctcaccgtggacaagagcaggtggcaggaggggaatgtcttctcatgctccgtgatgcatgaggctctgcacaaccactacacacagaagtccctctccctgtctctgggtaaatga

SEQ ID NO: 208 - protein, 448 aa, Homo sapiens
QVQLQQSGPGLVKPSQTLSLTCAISGDSVSSNIAAWNWIRLSPSRGLEWLGRTFFRSTWFYDYSLSVKGRITINPDTSKNQFSLHLNSVTPEDAAVYYCARTGRRWSLDYWGQGTLVTVSSASTKGPSVFPLAPCSRSTSESTAALGCLVKDYFPEPVTVSWNSGALTSGVHTFPAVLQSSGLYSLSSVVTVPSSSLGTKTYTCNVDHKPSNTKVDKRVESKYGPPCPPCPAPEFLGGPSVFLFPPKPKDTLMISRTPEVTCVVVDVSQEDPEVQFNWYVDGVEVHNAKTKPREEQFNSTYRVVSVLTVLHQDWLNGKEYKCKVSNKGLPSSIEKTISKAKGQPREPQVYTLPPSQEEMTKNQVSLTCLVKGFYPSDIAVEWESNGQPENNYKTTPPVLDSDGSFFLYSRLTVDKSRWQEGNVFSCSVMHEALHNHYTQKSLSLSLGK

SEQ ID NO: 209 - DNA, 348 bp, Homo sapiens
  source 1..348: mol_type = other DNA
gaggtgcagctggtggagtctgggggaggtgtggtacggcctggggggtccctgagactctcctgtgcaacctctggattcacctttgatgattatggcatgagctgggtccgccaagttccagggaaggggctggagtgggtctctagtgttaataggaatggtggtaccacagattatgcagactctgtgaagggccgattcaccatctccagagacaatgccaagaggtccctttttctgcaaatgaatagtctgagagccgaagacacggccttgtatcactgtgcgacaggggaacttttctttgactattggggccagggaaccctggtcaccgtctcctca

SEQ ID NO: 210 - protein, 116 aa, Homo sapiens
EVQLVESGGGVVRPGGSLRLSCATSGFTFDDYGMSWVRQVPGKGLEWVSSVNRNGGTTDYADSVKGRFTISRDNAKRSLFLQMNSLRAEDTALYHCATGELFFDYWGQGTLVTVSS

SEQ ID NO: 211 - DNA, 24 bp, Homo sapiens
  source 1..24: mol_type = other DNA
gttaataggaatggtggtaccaca

SEQ ID NO: 212 - protein, 8 aa, Homo sapiens
VNRNGGTT

SEQ ID NO: 213 - DNA, 27 bp, Homo sapiens
  source 1..27: mol_type = other DNA
gcgacaggggaacttttctttgactat

SEQ ID NO: 214 - protein, 9 aa, Homo sapiens
ATGELFFDY

SEQ ID NO: 215 - DNA, 1332 bp, Homo sapiens
  source 1..1332: mol_type = other DNA
gaggtgcagctggtggagtctgggggaggtgtggtacggcctggggggtccctgagactctcctgtgcaacctctggattcacctttgatgattatggcatgagctgggtccgccaagttccagggaaggggctggagtgggtctctagtgttaataggaatggtggtaccacagattatgcagactctgtgaagggccgattcaccatctccagagacaatgccaagaggtccctttttctgcaaatgaatagtctgagagccgaagacacggccttgtatcactgtgcgacaggggaacttttctttgactattggggccagggaaccctggtcaccgtctcctcagcctccaccaagggcccatcggtcttccccctggcgccctgctccaggagcacctccgagagcacagccgccctgggctgcctggtcaaggactacttccccgaaccggtgacggtgtcgtggaactcaggcgccctgaccagcggcgtgcacaccttcccggctgtcctacagtcctcaggactctactccctcagcagcgtggtgaccgtgccctccagcagcttgggcacgaagacctacacctgcaacgtagatcacaagcccagcaacaccaaggtggacaagagagttgagtccaaatatggtcccccatgcccaccctgcccagcacctgagttcctggggggaccatcagtcttcctgttccccccaaaacccaaggacactctcatgatctcccggacccctgaggtcacgtgcgtggtggtggacgtgagccaggaagaccccgaggtccagttcaactggtacgtggatggcgtggaggtgcataatgccaagacaaagccgcgggaggagcagttcaacagcacgtaccgtgtggtcagcgtcctcaccgtcctgcaccaggactggctgaacggcaaggagtacaagtgcaaggtctccaacaaaggcctcccgtcctccatcgagaaaaccatctccaaagccaaagggcagccccgagagccacaggtgtacaccctgcccccatcccaggaggagatgaccaagaaccaggtcagcctgacctgcctggtcaaaggcttctaccccagcgacatcgccgtggagtgggagagcaatgggcagccggagaacaactacaagaccacgcctcccgtgctggactccgacggctccttcttcctctacagcaggctcaccgtggacaagagcaggtggcaggaggggaatgtcttctcatgctccgtgatgcatgaggctctgcacaaccactacacacagaagtccctctccctgtctctgggtaaatga

SEQ ID NO: 216 - protein, 443 aa, Homo sapiens
EVQLVESGGGVVRPGGSLRLSCATSGFTFDDYGMSWVRQVPGKGLEWVSSVNRNGGTTDYADSVKGRFTISRDNAKRSLFLQMNSLRAEDTALYHCATGELFFDYWGQGTLVTVSSASTKGPSVFPLAPCSRSTSESTAALGCLVKDYFPEPVTVSWNSGALTSGVHTFPAVLQSSGLYSLSSVVTVPSSSLGTKTYTCNVDHKPSNTKVDKRVESKYGPPCPPCPAPEFLGGPSVFLFPPKPKDTLMISRTPEVTCVVVDVSQEDPEVQFNWYVDGVEVHNAKTKPREEQFNSTYRVVSVLTVLHQDWLNGKEYKCKVSNKGLPSSIEKTISKAKGQPREPQVYTLPPSQEEMTKNQVSLTCLVKGFYPSDIAVEWESNGQPENNYKTTPPVLDSDGSFFLYSRLTVDKSRWQEGNVFSCSVMHEALHNHYTQKSLSLSLGK

SEQ ID NO: 217 - DNA, 357 bp, Homo sapiens
  source 1..357: mol_type = other DNA
caggtccagctggtacagtctggggctgaggtgaagaagcctggggcctcagtgaaggtctcctgcaaggcttctggatacaccttcaccggccactatatgcactgggtgcgacaggcccctggacaagggcttgagtggatgggatggatctaccctcacagtggtcacacaaattatgcaaagaggtttcagggcagggtcaccatgaccagggacacgtccatcactacagcctacatggagctgatcaggctgagatctgacgacacggccgtgtattactgtgcgagaaggagtgggaggtcctggtatttcgatctgtggggccgtggcaccctggtcactgtctcctca

SEQ ID NO: 218 - protein, 119 aa, Homo sapiens
QVQLVQSGAEVKKPGASVKVSCKASGYTFTGHYMHWVRQAPGQGLEWMGWIYPHSGHTNYAKRFQGRVTMTRDTSITTAYMELIRLRSDDTAVYYCARRSGRSWYFDLWGRGTLVTVSS

SEQ ID NO: 219 - DNA, 24 bp, Homo sapiens
  source 1..24: mol_type = other DNA
ggatacaccttcaccggccactat

SEQ ID NO: 220 - protein, 8 aa, Homo sapiens
GYTFTGHY

SEQ ID NO: 221 - DNA, 24 bp, Homo sapiens
  source 1..24: mol_type = other DNA
atctaccctcacagtggtcacaca

SEQ ID NO: 222 - protein, 8 aa, Homo sapiens
IYPHSGHT

SEQ ID NO: 223 - DNA, 36 bp, Homo sapiens
  source 1..36: mol_type = other DNA
gcgagaaggagtgggaggtcctggtatttcgatctg

SEQ ID NO: 224 - protein, 12 aa, Homo sapiens
ARRSGRSWYFDL

SEQ ID NO: 225 - DNA, 324 bp, Homo sapiens
  source 1..324: mol_type = other DNA
gaaatagttttgacacagagtcccggcacactgtcactctctcccggggaaagagccaccttgtcatgtagagcaagtcagtcagtctctagctcttatctcgcctggtaccagcagaagccgggacaggcccctagactgctgatctacggggcaagttccagggccaccggaatccccgaccggttcagtggaagcggaagcggaaccgattttactttgacgatttctagactggagccagaggatttcgccgtttactattgtcaacagtacggaagcagcccgtggacgtttggccagggcacgaaggtagaaatcaag

SEQ ID NO: 226 - protein, 108 aa, Homo sapiens
EIVLTQSPGTLSLSPGERATLSCRASQSVSSSYLAWYQQKPGQAPRLLIYGASSRATGIPDRFSGSGSGTDFTLTISRLEPEDFAVYYCQQYGSSPWTFGQGTKVEIK

SEQ ID NO: 227 - DNA, 21 bp, Homo sapiens
  source 1..21: mol_type = other DNA
cagtcagtctctagctcttat

SEQ ID NO: 228 - protein, 7 aa, Homo sapiens
QSVSSSY

SEQ ID NO: 229-230 - skipped (2 entries)

SEQ ID NO: 231 - DNA, 27 bp, Homo sapiens
  source 1..27: mol_type = other DNA
caacagtacggaagcagcccgtggacg

SEQ ID NO: 232 - protein, 9 aa, Homo sapiens
QQYGSSPWT

SEQ ID NO: 233 - DNA, 1341 bp, Homo sapiens
  source 1..1341: mol_type = other DNA
caggtccagctggtacagtctggggctgaggtgaagaagcctggggcctcagtgaaggtctcctgcaaggcttctggatacaccttcaccggccactatatgcactgggtgcgacaggcccctggacaagggcttgagtggatgggatggatctaccctcacagtggtcacacaaattatgcaaagaggtttcagggcagggtcaccatgaccagggacacgtccatcactacagcctacatggagctgatcaggctgagatctgacgacacggccgtgtattactgtgcgagaaggagtgggaggtcctggtatttcgatctgtggggccgtggcaccctggtcactgtctcctcagcctccaccaagggcccatcggtcttccccctggcgccctgctccaggagcacctccgagagcacagccgccctgggctgcctggtcaaggactacttccccgaaccggtgacggtgtcgtggaactcaggcgccctgaccagcggcgtgcacaccttcccggctgtcctacagtcctcaggactctactccctcagcagcgtggtgaccgtgccctccagcagcttgggcacgaagacctacacctgcaacgtagatcacaagcccagcaacaccaaggtggacaagagagttgagtccaaatatggtcccccatgcccaccctgcccagcacctgagttcctggggggaccatcagtcttcctgttccccccaaaacccaaggacactctcatgatctcccggacccctgaggtcacgtgcgtggtggtggacgtgagccaggaagaccccgaggtccagttcaactggtacgtggatggcgtggaggtgcataatgccaagacaaagccgcgggaggagcagttcaacagcacgtaccgtgtggtcagcgtcctcaccgtcctgcaccaggactggctgaacggcaaggagtacaagtgcaaggtctccaacaaaggcctcccgtcctccatcgagaaaaccatctccaaagccaaagggcagccccgagagccacaggtgtacaccctgcccccatcccaggaggagatgaccaagaaccaggtcagcctgacctgcctggtcaaaggcttctaccccagcgacatcgccgtggagtgggagagcaatgggcagccggagaacaactacaagaccacgcctcccgtgctggactccgacggctccttcttcctctacagcaggctcaccgtggacaagagcaggtggcaggaggggaatgtcttctcatgctccgtgatgcatgaggctctgcacaaccactacacacagaagtccctctccctgtctctgggtaaatga

SEQ ID NO: 234 - protein, 446 aa, Homo sapiens
QVQLVQSGAEVKKPGASVKVSCKASGYTFTGHYMHWVRQAPGQGLEWMGWIYPHSGHTNYAKRFQGRVTMTRDTSITTAYMELIRLRSDDTAVYYCARRSGRSWYFDLWGRGTLVTVSSASTKGPSVFPLAPCSRSTSESTAALGCLVKDYFPEPVTVSWNSGALTSGVHTFPAVLQSSGLYSLSSVVTVPSSSLGTKTYTCNVDHKPSNTKVDKRVESKYGPPCPPCPAPEFLGGPSVFLFPPKPKDTLMISRTPEVTCVVVDVSQEDPEVQFNWYVDGVEVHNAKTKPREEQFNSTYRVVSVLTVLHQDWLNGKEYKCKVSNKGLPSSIEKTISKAKGQPREPQVYTLPPSQEEMTKNQVSLTCLVKGFYPSDIAVEWESNGQPENNYKTTPPVLDSDGSFFLYSRLTVDKSRWQEGNVFSCSVMHEALHNHYTQKSLSLSLGK

SEQ ID NO: 235 - DNA, 648 bp, Homo sapiens
  source 1..648: mol_type = other DNA
gaaatagttttgacacagagtcccggcacactgtcactctctcccggggaaagagccaccttgtcatgtagagcaagtcagtcagtctctagctcttatctcgcctggtaccagcagaagccgggacaggcccctagactgctgatctacggggcaagttccagggccaccggaatccccgaccggttcagtggaagcggaagcggaaccgattttactttgacgatttctagactggagccagaggatttcgccgtttactattgtcaacagtacggaagcagcccgtggacgtttggccagggcacgaaggtagaaatcaagcgaactgtggctgcaccatctgtcttcatcttcccgccatctgatgagcagttgaaatctggaactgcctctgttgtgtgcctgctgaataacttctatcccagagaggccaaagtacagtggaaggtggataacgccctccaatcgggtaactcccaggagagtgtcacagagcaggacagcaaggacagcacctacagcctcagcagcaccctgacgctgagcaaagcagactacgagaaacacaaagtctacgcctgcgaagtcacccatcagggcctgagctcgcccgtcacaaagagcttcaacaggggagagtgttag

SEQ ID NO: 236 - protein, 215 aa, Homo sapiens
EIVLTQSPGTLSLSPGERATLSCRASQSVSSSYLAWYQQKPGQAPRLLIYGASSRATGIPDRFSGSGSGTDFTLTISRLEPEDFAVYYCQQYGSSPWTFGQGTKVEIKRTVAAPSVFIFPPSDEQLKSGTASVVCLLNNFYPREAKVQWKVDNALQSGNSQESVTEQDSKDSTYSLSSTLTLSKADYEKHKVYACEVTHQGLSSPVTKSFNRGEC

SEQ ID NO: 237 - DNA, 351 bp, Homo sapiens
  source 1..351: mol_type = other DNA
gaggtgcagctggtggagtctgggggagggttggtacagcctggggggtccctgggactctcctgtgcagcctctggattcacctttagcaactatgccatgagctgggtccgccaggctccagggaaggggctggagtgggtctcagctgttagtggtggtggtggtggcacatactacgcagactccgtgaagggccggttcaccatctccagagacaattccaagaacacggttcttctgcaaatgaacagcctgagagccgaggacacggccgtatattactgtgcgagaggtcggactgggggccttgactactggggcccgggaaccctggtcaccgtctcctca

SEQ ID NO: 238 - protein, 117 aa, Homo sapiens
EVQLVESGGGLVQPGGSLGLSCAASGFTFSNYAMSWVRQAPGKGLEWVSAVSGGGGGTYYADSVKGRFTISRDNSKNTVLLQMNSLRAEDTAVYYCARGRTGGLDYWGPGTLVTVSS

SEQ ID NO: 239 - DNA, 24 bp, Homo sapiens
  source 1..24: mol_type = other DNA
ggattcacctttagcaactatgcc

SEQ ID NO: 240 - protein, 8 aa, Homo sapiens
GFTFSNYA

SEQ ID NO: 241 - DNA, 24 bp, Homo sapiens
  source 1..24: mol_type = other DNA
gttagtggtggtggtggtggcaca

SEQ ID NO: 242 - protein, 8 aa, Homo sapiens
VSGGGGGT

SEQ ID NO: 243 - DNA, 30 bp, Homo sapiens
  source 1..30: mol_type = other DNA
gcgagaggtcggactgggggccttgactac

SEQ ID NO: 244 - protein, 10 aa, Homo sapiens
ARGRTGGLDY

SEQ ID NO: 245 - DNA, 336 bp, Homo sapiens
  source 1..336: mol_type = other DNA
gatgttgtgatgactcagtctcctctctccctgcccgtcatctttggacagccggcctccatctcctgcaggtcaagtcaaagcctcgtagacagtgatggaaacacctacttgaattggcttcagcagaggccaggccaatctccaaggcgcctaatttatgaggtttctaaccgggactctggggtcccagacagattcagcggcagtgggtcaggcactgatttcacactgacaatcagcagggtggaggctgaggatgttggcatttattactgcatgcaaggtacgcgctggcctcctactttcggcggagggaccaaggtggagatcaaa

SEQ ID NO: 246 - protein, 112 aa, Homo sapiens
DVVMTQSPLSLPVIFGQPASISCRSSQSLVDSDGNTYLNWLQQRPGQSPRRLIYEVSNRDSGVPDRFSGSGSGTDFTLTISRVEAEDVGIYYCMQGTRWPPTFGGGTKVEIK

SEQ ID NO: 247 - DNA, 33 bp, Homo sapiens
  source 1..33: mol_type = other DNA
caaagcctcgtagacagtgatggaaacacctac

SEQ ID NO: 248 - protein, 11 aa, Homo sapiens
QSLVDSDGNTY

SEQ ID NO: 249-250 - skipped (2 entries)

SEQ ID NO: 251 - DNA, 27 bp, Homo sapiens
  source 1..27: mol_type = other DNA
atgcaaggtacgcgctggcctcctact

SEQ ID NO: 252 - protein, 9 aa, Homo sapiens
MQGTRWPPT

SEQ ID NO: 253 - DNA, 1335 bp, Homo sapiens
  source 1..1335: mol_type = other DNA
gaggtgcagctggtggagtctgggggagggttggtacagcctggggggtccctgggactctcctgtgcagcctctggattcacctttagcaactatgccatgagctgggtccgccaggctccagggaaggggctggagtgggtctcagctgttagtggtggtggtggtggcacatactacgcagactccgtgaagggccggttcaccatctccagagacaattccaagaacacggttcttctgcaaatgaacagcctgagagccgaggacacggccgtatattactgtgcgagaggtcggactgggggccttgactactggggcccgggaaccctggtcaccgtctcctcagcctccaccaagggcccatcggtcttccccctggcgccctgctccaggagcacctccgagagcacagccgccctgggctgcctggtcaaggactacttccccgaaccggtgacggtgtcgtggaactcaggcgccctgaccagcggcgtgcacaccttcccggctgtcctacagtcctcaggactctactccctcagcagcgtggtgaccgtgccctccagcagcttgggcacgaagacctacacctgcaacgtagatcacaagcccagcaacaccaaggtggacaagagagttgagtccaaatatggtcccccatgcccaccctgcccagcacctgagttcctggggggaccatcagtcttcctgttccccccaaaacccaaggacactctcatgatctcccggacccctgaggtcacgtgcgtggtggtggacgtgagccaggaagaccccgaggtccagttcaactggtacgtggatggcgtggaggtgcataatgccaagacaaagccgcgggaggagcagttcaacagcacgtaccgtgtggtcagcgtcctcaccgtcctgcaccaggactggctgaacggcaaggagtacaagtgcaaggtctccaacaaaggcctcccgtcctccatcgagaaaaccatctccaaagccaaagggcagccccgagagccacaggtgtacaccctgcccccatcccaggaggagatgaccaagaaccaggtcagcctgacctgcctggtcaaaggcttctaccccagcgacatcgccgtggagtgggagagcaatgggcagccggagaacaactacaagaccacgcctcccgtgctggactccgacggctccttcttcctctacagcaggctcaccgtggacaagagcaggtggcaggaggggaatgtcttctcatgctccgtgatgcatgaggctctgcacaaccactacacacagaagtccctctccctgtctctgggtaaatga

SEQ ID NO: 254 - protein, 444 aa, Homo sapiens
EVQLVESGGGLVQPGGSLGLSCAASGFTFSNYAMSWVRQAPGKGLEWVSAVSGGGGGTYYADSVKGRFTISRDNSKNTVLLQMNSLRAEDTAVYYCARGRTGGLDYWGPGTLVTVSSASTKGPSVFPLAPCSRSTSESTAALGCLVKDYFPEPVTVSWNSGALTSGVHTFPAVLQSSGLYSLSSVVTVPSSSLGTKTYTCNVDHKPSNTKVDKRVESKYGPPCPPCPAPEFLGGPSVFLFPPKPKDTLMISRTPEVTCVVVDVSQEDPEVQFNWYVDGVEVHNAKTKPREEQFNSTYRVVSVLTVLHQDWLNGKEYKCKVSNKGLPSSIEKTISKAKGQPREPQVYTLPPSQEEMTKNQVSLTCLVKGFYPSDIAVEWESNGQPENNYKTTPPVLDSDGSFFLYSRLTVDKSRWQEGNVFSCSVMHEALHNHYTQKSLSLSLGK

SEQ ID NO: 255 - DNA, 660 bp, Homo sapiens
  source 1..660: mol_type = other DNA
gatgttgtgatgactcagtctcctctctccctgcccgtcatctttggacagccggcctccatctcctgcaggtcaagtcaaagcctcgtagacagtgatggaaacacctacttgaattggcttcagcagaggccaggccaatctccaaggcgcctaatttatgaggtttctaaccgggactctggggtcccagacagattcagcggcagtgggtcaggcactgatttcacactgacaatcagcagggtggaggctgaggatgttggcatttattactgcatgcaaggtacgcgctggcctcctactttcggcggagggaccaaggtggagatcaaacgaactgtggctgcaccatctgtcttcatcttcccgccatctgatgagcagttgaaatctggaactgcctctgttgtgtgcctgctgaataacttctatcccagagaggccaaagtacagtggaaggtggataacgccctccaatcgggtaactcccaggagagtgtcacagagcaggacagcaaggacagcacctacagcctcagcagcaccctgacgctgagcaaagcagactacgagaaacacaaagtctacgcctgcgaagtcacccatcagggcctgagctcgcccgtcacaaagagcttcaacaggggagagtgttag

SEQ ID NO: 256 - protein, 219 aa, Homo sapiens
DVVMTQSPLSLPVIFGQPASISCRSSQSLVDSDGNTYLNWLQQRPGQSPRRLIYEVSNRDSGVPDRFSGSGSGTDFTLTISRVEAEDVGIYYCMQGTRWPPTFGGGTKVEIKRTVAAPSVFIFPPSDEQLKSGTASVVCLLNNFYPREAKVQWKVDNALQSGNSQESVTEQDSKDSTYSLSSTLTLSKADYEKHKVYACEVTHQGLSSPVTKSFNRGEC

SEQ ID NO: 257 - DNA, 366 bp, Homo sapiens
  source 1..366: mol_type = other DNA
gaggtgcagctggtggagtctgggggaggtgtggtccggcctggggggtccctgagactctcctgtgcagcctctggattcatctttgatgattatgacatgagttgggtccgccaacctccagggaggggactggaatgggtctccggtattgattggtttggtggtaccagaggttatgcagactctatgaagggccgattcaccatttccagagacaacgccaagaactccctgtatctgcaaatgaacagcctgagagtcgaggacacggccttctattactgtgcgagagggggggctatagtgggagctgttactccctttgactactggggccagggaaccctggtcactgtctcctca

SEQ ID NO: 258 - protein, 122 aa, Homo sapiens
EVQLVESGGGVVRPGGSLRLSCAASGFIFDDYDMSWVRQPPGRGLEWVSGIDWFGGTRGYADSMKGRFTISRDNAKNSLYLQMNSLRVEDTAFYYCARGGAIVGAVTPFDYWGQGTLVTVSS

SEQ ID NO: 259 - DNA, 24 bp, Homo sapiens
  source 1..24: mol_type = other DNA
ggattcatctttgatgattatgac

SEQ ID NO: 260 - protein, 8 aa, Homo sapiens
GFIFDDYD

SEQ ID NO: 261 - DNA, 24 bp, Homo sapiens
  source 1..24: mol_type = other DNA
attgattggtttggtggtaccaga

SEQ ID NO: 262 - protein, 8 aa, Homo sapiens
IDWFGGTR

SEQ ID NO: 263 - DNA, 45 bp, Homo sapiens
  source 1..45: mol_type = other DNA
gcgagagggggggctatagtgggagctgttactccctttgactac

SEQ ID NO: 264 - protein, 15 aa, Homo sapiens
ARGGAIVGAVTPFDY

SEQ ID NO: 265 - DNA, 321 bp, Homo sapiens
  source 1..321: mol_type = other DNA
gacatccagatgacccagtctccatcctccctgtctgcatctgttggaaacagagtcaccctcagttgccgggcaagtcagagcattaacacctatttaagttggtatcagcagagaccaggaaaagcccctaagctcctgatctatgctgcatccagtttgcaaagtggggtcccctcaaggttcagtggcagtggagctgggacagatttcactctcaccatcagcagtctgcaacctgaagattttgcaacttactactgtcaacagagttacagtgcccctctcactttcggcggtgggaccaaggtggagatcaaa

SEQ ID NO: 266 - protein, 107 aa, Homo sapiens
DIQMTQSPSSLSASVGNRVTLSCRASQSINTYLSWYQQRPGKAPKLLIYAASSLQSGVPSRFSGSGAGTDFTLTISSLQPEDFATYYCQQSYSAPLTFGGGTKVEIK

SEQ ID NO: 267 - DNA, 18 bp, Homo sapiens
  source 1..18: mol_type = other DNA
cagagcattaacacctat

SEQ ID NO: 268 - protein, 6 aa, Homo sapiens
QSINTY

SEQ ID NO: 269 - DNA, 27 bp, Homo sapiens
  source 1..27: mol_type = other DNA
caacagagttacagtgcccctctcact

SEQ ID NO: 270 - protein, 9 aa, Homo sapiens
QQSYSAPLT

SEQ ID NO: 271 - DNA, 1350 bp, Homo sapiens
  source 1..1350: mol_type = other DNA
gaggtgcagctggtggagtctgggggaggtgtggtccggcctggggggtccctgagactctcctgtgcagcctctggattcatctttgatgattatgacatgagttgggtccgccaacctccagggaggggactggaatgggtctccggtattgattggtttggtggtaccagaggttatgcagactctatgaagggccgattcaccatttccagagacaacgccaagaactccctgtatctgcaaatgaacagcctgagagtcgaggacacggccttctattactgtgcgagagggggggctatagtgggagctgttactccctttgactactggggccagggaaccctggtcactgtctcctcagcctccaccaagggcccatcggtcttccccctggcgccctgctccaggagcacctccgagagcacagccgccctgggctgcctggtcaaggactacttccccgaaccggtgacggtgtcgtggaactcaggcgccctgaccagcggcgtgcacaccttcccggctgtcctacagtcctcaggactctactccctcagcagcgtggtgaccgtgccctccagcagcttgggcacgaagacctacacctgcaacgtagatcacaagcccagcaacaccaaggtggacaagagagttgagtccaaatatggtcccccatgcccaccctgcccagcacctgagttcctggggggaccatcagtcttcctgttccccccaaaacccaaggacactctcatgatctcccggacccctgaggtcacgtgcgtggtggtggacgtgagccaggaagaccccgaggtccagttcaactggtacgtggatggcgtggaggtgcataatgccaagacaaagccgcgggaggagcagttcaacagcacgtaccgtgtggtcagcgtcctcaccgtcctgcaccaggactggctgaacggcaaggagtacaagtgcaaggtctccaacaaaggcctcccgtcctccatcgagaaaaccatctccaaagccaaagggcagccccgagagccacaggtgtacaccctgcccccatcccaggaggagatgaccaagaaccaggtcagcctgacctgcctggtcaaaggcttctaccccagcgacatcgccgtggagtgggagagcaatgggcagccggagaacaactacaagaccacgcctcccgtgctggactccgacggctccttcttcctctacagcaggctcaccgtggacaagagcaggtggcaggaggggaatgtcttctcatgctccgtgatgcatgaggctctgcacaaccactacacacagaagtccctctccctgtctctgggtaaatga

SEQ ID NO: 272 - protein, 449 aa, Homo sapiens
EVQLVESGGGVVRPGGSLRLSCAASGFIFDDYDMSWVRQPPGRGLEWVSGIDWFGGTRGYADSMKGRFTISRDNAKNSLYLQMNSLRVEDTAFYYCARGGAIVGAVTPFDYWGQGTLVTVSSASTKGPSVFPLAPCSRSTSESTAALGCLVKDYFPEPVTVSWNSGALTSGVHTFPAVLQSSGLYSLSSVVTVPSSSLGTKTYTCNVDHKPSNTKVDKRVESKYGPPCPPCPAPEFLGGPSVFLFPPKPKDTLMISRTPEVTCVVVDVSQEDPEVQFNWYVDGVEVHNAKTKPREEQFNSTYRVVSVLTVLHQDWLNGKEYKCKVSNKGLPSSIEKTISKAKGQPREPQVYTLPPSQEEMTKNQVSLTCLVKGFYPSDIAVEWESNGQPENNYKTTPPVLDSDGSFFLYSRLTVDKSRWQEGNVFSCSVMHEALHNHYTQKSLSLSLGK

SEQ ID NO: 273 - DNA, 645 bp, Homo sapiens
  source 1..645: mol_type = other DNA
gacatccagatgacccagtctccatcctccctgtctgcatctgttggaaacagagtcaccctcagttgccgggcaagtcagagcattaacacctatttaagttggtatcagcagagaccaggaaaagcccctaagctcctgatctatgctgcatccagtttgcaaagtggggtcccctcaaggttcagtggcagtggagctgggacagatttcactctcaccatcagcagtctgcaacctgaagattttgcaacttactactgtcaacagagttacagtgcccctctcactttcggcggtgggaccaaggtggagatcaaacgaactgtggctgcaccatctgtcttcatcttcccgccatctgatgagcagttgaaatctggaactgcctctgttgtgtgcctgctgaataacttctatcccagagaggccaaagtacagtggaaggtggataacgccctccaatcgggtaactcccaggagagtgtcacagagcaggacagcaaggacagcacctacagcctcagcagcaccctgacgctgagcaaagcagactacgagaaacacaaagtctacgcctgcgaagtcacccatcagggcctgagctcgcccgtcacaaagagcttcaacaggggagagtgttag

SEQ ID NO: 274 - protein, 214 aa, Homo sapiens
DIQMTQSPSSLSASVGNRVTLSCRASQSINTYLSWYQQRPGKAPKLLIYAASSLQSGVPSRFSGSGAGTDFTLTISSLQPEDFATYYCQQSYSAPLTFGGGTKVEIKRTVAAPSVFIFPPSDEQLKSGTASVVCLLNNFYPREAKVQWKVDNALQSGNSQESVTEQDSKDSTYSLSSTLTLSKADYEKHKVYACEVTHQGLSSPVTKSFNRGEC

SEQ ID NO: 275 - DNA, 366 bp, Homo sapiens
  source 1..366: mol_type = other DNA
cagctgcagctgcaggagtcgggcccaggactggtgaagccttcggagaccctgtccctcacctgcactgtctctggtggctccatcagcattaagaattactactggggctggatccgtcagcccccagggaaggggctggagtggattgggagtatctattatagtgggaccacctactacaacccgtccctcaagagtcgagtcaccatatccgtagacacgtccaagaaccagttctccctgaagctgagctctgtgaccgccgcagacacggctgtatatcactgtgcgagacatggatacagctatggtcacggctggttcgacccctggggccagggaaccctggtcaccgtctcctca

SEQ ID NO: 276 - protein, 122 aa, Homo sapiens
QLQLQESGPGLVKPSETLSLTCTVSGGSISIKNYYWGWIRQPPGKGLEWIGSIYYSGTTYYNPSLKSRVTISVDTSKNQFSLKLSSVTAADTAVYHCARHGYSYGHGWFDPWGQGTLVTVSS

SEQ ID NO: 277 - DNA, 30 bp, Homo sapiens
  source 1..30: mol_type = other DNA
ggtggctccatcagcattaagaattactac

SEQ ID NO: 278 - protein, 10 aa, Homo sapiens
GGSISIKNYY

SEQ ID NO: 279 - DNA, 21 bp, Homo sapiens
  source 1..21: mol_type = other DNA
atctattatagtgggaccacc

SEQ ID NO: 280 - protein, 7 aa, Homo sapiens
IYYSGTT

SEQ ID NO: 281 - DNA, 42 bp, Homo sapiens
  source 1..42: mol_type = other DNA
gcgagacatggatacagctatggtcacggctggttcgacccc

SEQ ID NO: 282 - protein, 14 aa, Homo sapiens
ARHGYSYGHGWFDP

SEQ ID NO: 283 - DNA, 1350 bp, Homo sapiens
  source 1..1350: mol_type = other DNA
cagctgcagctgcaggagtcgggcccaggactggtgaagccttcggagaccctgtccctcacctgcactgtctctggtggctccatcagcattaagaattactactggggctggatccgtcagcccccagggaaggggctggagtggattgggagtatctattatagtgggaccacctactacaacccgtccctcaagagtcgagtcaccatatccgtagacacgtccaagaaccagttctccctgaagctgagctctgtgaccgccgcagacacggctgtatatcactgtgcgagacatggatacagctatggtcacggctggttcgacccctggggccagggaaccctggtcaccgtctcctcagcctccaccaagggcccatcggtcttccccctggcgccctgctccaggagcacctccgagagcacagccgccctgggctgcctggtcaaggactacttccccgaaccggtgacggtgtcgtggaactcaggcgccctgaccagcggcgtgcacaccttcccggctgtcctacagtcctcaggactctactccctcagcagcgtggtgaccgtgccctccagcagcttgggcacgaagacctacacctgcaacgtagatcacaagcccagcaacaccaaggtggacaagagagttgagtccaaatatggtcccccatgcccaccctgcccagcacctgagttcctggggggaccatcagtcttcctgttccccccaaaacccaaggacactctcatgatctcccggacccctgaggtcacgtgcgtggtggtggacgtgagccaggaagaccccgaggtccagttcaactggtacgtggatggcgtggaggtgcataatgccaagacaaagccgcgggaggagcagttcaacagcacgtaccgtgtggtcagcgtcctcaccgtcctgcaccaggactggctgaacggcaaggagtacaagtgcaaggtctccaacaaaggcctcccgtcctccatcgagaaaaccatctccaaagccaaagggcagccccgagagccacaggtgtacaccctgcccccatcccaggaggagatgaccaagaaccaggtcagcctgacctgcctggtcaaaggcttctaccccagcgacatcgccgtggagtgggagagcaatgggcagccggagaacaactacaagaccacgcctcccgtgctggactccgacggctccttcttcctctacagcaggctcaccgtggacaagagcaggtggcaggaggggaatgtcttctcatgctccgtgatgcatgaggctctgcacaaccactacacacagaagtccctctccctgtctctgggtaaatga

SEQ ID NO: 284 - protein, 449 aa, Homo sapiens
QLQLQESGPGLVKPSETLSLTCTVSGGSISIKNYYWGWIRQPPGKGLEWIGSIYYSGTTYYNPSLKSRVTISVDTSKNQFSLKLSSVTAADTAVYHCARHGYSYGHGWFDPWGQGTLVTVSSASTKGPSVFPLAPCSRSTSESTAALGCLVKDYFPEPVTVSWNSGALTSGVHTFPAVLQSSGLYSLSSVVTVPSSSLGTKTYTCNVDHKPSNTKVDKRVESKYGPPCPPCPAPEFLGGPSVFLFPPKPKDTLMISRTPEVTCVVVDVSQEDPEVQFNWYVDGVEVHNAKTKPREEQFNSTYRVVSVLTVLHQDWLNGKEYKCKVSNKGLPSSIEKTISKAKGQPREPQVYTLPPSQEEMTKNQVSLTCLVKGFYPSDIAVEWESNGQPENNYKTTPPVLDSDGSFFLYSRLTVDKSRWQEGNVFSCSVMHEALHNHYTQKSLSLSLGK

SEQ ID NO: 285 - DNA, 366 bp, Homo sapiens
  source 1..366: mol_type = other DNA
caggtacagctgcagcagtcaggtccaggactggtaaagccctcacagaccctctcactcacctgtgacatctccggggacagtgtctctagcaacattgctacttggaactggatcaggcagtccccatcgagaggccttgagtggctgggaaggacatattacaggtccaagtggtataaagattatgcagtatctgtgaaaagtcgaataaccatcaacccagacacatccaagaaccagttctccctgcaggtgaactctgtgactcccgaggacacggctgtctattactgtgcaagaatgactgggccgcgatactactttgagtactggggccagggaaccctggtcaccgtctcctca

SEQ ID NO: 286 - protein, 122 aa, Homo sapiens
QVQLQQSGPGLVKPSQTLSLTCDISGDSVSSNIATWNWIRQSPSRGLEWLGRTYYRSKWYKDYAVSVKSRITINPDTSKNQFSLQVNSVTPEDTAVYYCARMTGPRYYFEYWGQGTLVTVSS

SEQ ID NO: 287 - DNA, 30 bp, Homo sapiens
  source 1..30: mol_type = other DNA
ggggacagtgtctctagcaacattgctact

SEQ ID NO: 288 - protein, 10 aa, Homo sapiens
GDSVSSNIAT

SEQ ID NO: 289 - DNA, 27 bp, Homo sapiens
  source 1..27: mol_type = other DNA
acatattacaggtccaagtggtataaa

SEQ ID NO: 290 - protein, 9 aa, Homo sapiens
TYYRSKWYK

SEQ ID NO: 291 - DNA, 36 bp, Homo sapiens
  source 1..36: mol_type = other DNA
gcaagaatgactgggccgcgatactactttgagtac

SEQ ID NO: 292 - protein, 12 aa, Homo sapiens
ARMTGPRYYFEY

SEQ ID NO: 293 - DNA, 1350 bp, Homo sapiens
  source 1..1350: mol_type = other DNA
caggtacagctgcagcagtcaggtccaggactggtaaagccctcacagaccctctcactcacctgtgacatctccggggacagtgtctctagcaacattgctacttggaactggatcaggcagtccccatcgagaggccttgagtggctgggaaggacatattacaggtccaagtggtataaagattatgcagtatctgtgaaaagtcgaataaccatcaacccagacacatccaagaaccagttctccctgcaggtgaactctgtgactcccgaggacacggctgtctattactgtgcaagaatgactgggccgcgatactactttgagtactggggccagggaaccctggtcaccgtctcctcagcctccaccaagggcccatcggtcttccccctggcgccctgctccaggagcacctccgagagcacagccgccctgggctgcctggtcaaggactacttccccgaaccggtgacggtgtcgtggaactcaggcgccctgaccagcggcgtgcacaccttcccggctgtcctacagtcctcaggactctactccctcagcagcgtggtgaccgtgccctccagcagcttgggcacgaagacctacacctgcaacgtagatcacaagcccagcaacaccaaggtggacaagagagttgagtccaaatatggtcccccatgcccaccctgcccagcacctgagttcctggggggaccatcagtcttcctgttccccccaaaacccaaggacactctcatgatctcccggacccctgaggtcacgtgcgtggtggtggacgtgagccaggaagaccccgaggtccagttcaactggtacgtggatggcgtggaggtgcataatgccaagacaaagccgcgggaggagcagttcaacagcacgtaccgtgtggtcagcgtcctcaccgtcctgcaccaggactggctgaacggcaaggagtacaagtgcaaggtctccaacaaaggcctcccgtcctccatcgagaaaaccatctccaaagccaaagggcagccccgagagccacaggtgtacaccctgcccccatcccaggaggagatgaccaagaaccaggtcagcctgacctgcctggtcaaaggcttctaccccagcgacatcgccgtggagtgggagagcaatgggcagccggagaacaactacaagaccacgcctcccgtgctggactccgacggctccttcttcctctacagcaggctcaccgtggacaagagcaggtggcaggaggggaatgtcttctcatgctccgtgatgcatgaggctctgcacaaccactacacacagaagtccctctccctgtctctgggtaaatga

SEQ ID NO: 294 - protein, 449 aa, Homo sapiens
QVQLQQSGPGLVKPSQTLSLTCDISGDSVSSNIATWNWIRQSPSRGLEWLGRTYYRSKWYKDYAVSVKSRITINPDTSKNQFSLQVNSVTPEDTAVYYCARMTGPRYYFEYWGQGTLVTVSSASTKGPSVFPLAPCSRSTSESTAALGCLVKDYFPEPVTVSWNSGALTSGVHTFPAVLQSSGLYSLSSVVTVPSSSLGTKTYTCNVDHKPSNTKVDKRVESKYGPPCPPCPAPEFLGGPSVFLFPPKPKDTLMISRTPEVTCVVVDVSQEDPEVQFNWYVDGVEVHNAKTKPREEQFNSTYRVVSVLTVLHQDWLNGKEYKCKVSNKGLPSSIEKTISKAKGQPREPQVYTLPPSQEEMTKNQVSLTCLVKGFYPSDIAVEWESNGQPENNYKTTPPVLDSDGSFFLYSRLTVDKSRWQEGNVFSCSVMHEALHNHYTQKSLSLSLGK

SEQ ID NO: 295 - DNA, 366 bp, Homo sapiens
  source 1..366: mol_type = other DNA
gaggtgcagctggtggagtctgggggaggtgtggtccggcctggggggtccctgagactctcctgtgcagcctctggattcacctttgatgattttgacatgagctgggtccgccaaggtccagggaaggggctggagtgggtctctggtattaattggcatgggagtagtacaggttatgcagactctgtgaagggccgattcaccatctccagagacaacgccaagaactccctgtatctgcaaatgagcagtctgagggccgaggacacggccttatatcactgtgtgagaggggggactatagtgggtgccactactccccttgactactggggccagggaaccctggtcaccgtctcctca

SEQ ID NO: 296 - protein, 122 aa, Homo sapiens
EVQLVESGGGVVRPGGSLRLSCAASGFTFDDFDMSWVRQGPGKGLEWVSGINWHGSSTGYADSVKGRFTISRDNAKNSLYLQMSSLRAEDTALYHCVRGGTIVGATTPLDYWGQGTLVTVSS

SEQ ID NO: 297 - DNA, 24 bp, Homo sapiens
  source 1..24: mol_type = other DNA
ggattcacctttgatgattttgac

SEQ ID NO: 298 - protein, 8 aa, Homo sapiens
GFTFDDFD

SEQ ID NO: 299 - DNA, 24 bp, Homo sapiens
  source 1..24: mol_type = other DNA
attaattggcatgggagtagtaca

SEQ ID NO: 300 - protein, 8 aa, Homo sapiens
INWHGSST

SEQ ID NO: 301 - DNA, 45 bp, Homo sapiens
  source 1..45: mol_type = other DNA
gtgagaggggggactatagtgggtgccactactccccttgactac

SEQ ID NO: 302 - protein, 15 aa, Homo sapiens
VRGGTIVGATTPLDY

SEQ ID NO: 303 - DNA, 321 bp, Homo sapiens
  source 1..321: mol_type = other DNA
gacatccagatgacccagtctccatcctccctgtctgcatctgtaggagacagagtcaccatgacttgccgggcaagtcggaccattagcagctatttaagttggtatcagcagaaatcagggaaagtccctaacctcctgatctttggtgcatccagtttgcaaagtggggtcccatcaaggttcagtgccagtggatctgggacagatttcactctcatcatcagcagtctgcaacctgaagattttgcaacttactactgtcaacagagttacagctcccctctcactttcggcggagggaccaaggtggagatcaaa

SEQ ID NO: 304 - protein, 107 aa, Homo sapiens
DIQMTQSPSSLSASVGDRVTMTCRASRTISSYLSWYQQKSGKVPNLLIFGASSLQSGVPSRFSASGSGTDFTLIISSLQPEDFATYYCQQSYSSPLTFGGGTKVEIK

SEQ ID NO: 305 - DNA, 18 bp, Homo sapiens
  source 1..18: mol_type = other DNA
cggaccattagcagctat

SEQ ID NO: 306 - protein, 6 aa, Homo sapiens
RTISSY

SEQ ID NO: 307 - skipped

SEQ ID NO: 308 - DNA, 27 bp, Homo sapiens
  source 1..27: mol_type = other DNA
caacagagttacagctcccctctcact

SEQ ID NO: 309 - protein, 9 aa, Homo sapiens
QQSYSSPLT

SEQ ID NO: 310 - DNA, 1350 bp, Homo sapiens
  source 1..1350: mol_type = other DNA
gaggtgcagctggtggagtctgggggaggtgtggtccggcctggggggtccctgagactctcctgtgcagcctctggattcacctttgatgattttgacatgagctgggtccgccaaggtccagggaaggggctggagtgggtctctggtattaattggcatgggagtagtacaggttatgcagactctgtgaagggccgattcaccatctccagagacaacgccaagaactccctgtatctgcaaatgagcagtctgagggccgaggacacggccttatatcactgtgtgagaggggggactatagtgggtgccactactccccttgactactggggccagggaaccctggtcaccgtctcctcagcctccaccaagggcccatcggtcttccccctggcgccctgctccaggagcacctccgagagcacagccgccctgggctgcctggtcaaggactacttccccgaaccggtgacggtgtcgtggaactcaggcgccctgaccagcggcgtgcacaccttcccggctgtcctacagtcctcaggactctactccctcagcagcgtggtgaccgtgccctccagcagcttgggcacgaagacctacacctgcaacgtagatcacaagcccagcaacaccaaggtggacaagagagttgagtccaaatatggtcccccatgcccaccctgcccagcacctgagttcctggggggaccatcagtcttcctgttccccccaaaacccaaggacactctcatgatctcccggacccctgaggtcacgtgcgtggtggtggacgtgagccaggaagaccccgaggtccagttcaactggtacgtggatggcgtggaggtgcataatgccaagacaaagccgcgggaggagcagttcaacagcacgtaccgtgtggtcagcgtcctcaccgtcctgcaccaggactggctgaacggcaaggagtacaagtgcaaggtctccaacaaaggcctcccgtcctccatcgagaaaaccatctccaaagccaaagggcagccccgagagccacaggtgtacaccctgcccccatcccaggaggagatgaccaagaaccaggtcagcctgacctgcctggtcaaaggcttctaccccagcgacatcgccgtggagtgggagagcaatgggcagccggagaacaactacaagaccacgcctcccgtgctggactccgacggctccttcttcctctacagcaggctcaccgtggacaagagcaggtggcaggaggggaatgtcttctcatgctccgtgatgcatgaggctctgcacaaccactacacacagaagtccctctccctgtctctgggtaaatga

SEQ ID NO: 311 - protein, 449 aa, Homo sapiens
EVQLVESGGGVVRPGGSLRLSCAASGFTFDDFDMSWVRQGPGKGLEWVSGINWHGSSTGYADSVKGRFTISRDNAKNSLYLQMSSLRAEDTALYHCVRGGTIVGATTPLDYWGQGTLVTVSSASTKGPSVFPLAPCSRSTSESTAALGCLVKDYFPEPVTVSWNSGALTSGVHTFPAVLQSSGLYSLSSVVTVPSSSLGTKTYTCNVDHKPSNTKVDKRVESKYGPPCPPCPAPEFLGGPSVFLFPPKPKDTLMISRTPEVTCVVVDVSQEDPEVQFNWYVDGVEVHNAKTKPREEQFNSTYRVVSVLTVLHQDWLNGKEYKCKVSNKGLPSSIEKTISKAKGQPREPQVYTLPPSQEEMTKNQVSLTCLVKGFYPSDIAVEWESNGQPENNYKTTPPVLDSDGSFFLYSRLTVDKSRWQEGNVFSCSVMHEALHNHYTQKSLSLSLGK

SEQ ID NO: 312 - DNA, 645 bp, Homo sapiens
  source 1..645: mol_type = other DNA
gacatccagatgacccagtctccatcctccctgtctgcatctgtaggagacagagtcaccatgacttgccgggcaagtcggaccattagcagctatttaagttggtatcagcagaaatcagggaaagtccctaacctcctgatctttggtgcatccagtttgcaaagtggggtcccatcaaggttcagtgccagtggatctgggacagatttcactctcatcatcagcagtctgcaacctgaagattttgcaacttactactgtcaacagagttacagctcccctctcactttcggcggagggaccaaggtggagatcaaacgaactgtggctgcaccatctgtcttcatcttcccgccatctgatgagcagttgaaatctggaactgcctctgttgtgtgcctgctgaataacttctatcccagagaggccaaagtacagtggaaggtggataacgccctccaatcgggtaactcccaggagagtgtcacagagcaggacagcaaggacagcacctacagcctcagcagcaccctgacgctgagcaaagcagactacgagaaacacaaagtctacgcctgcgaagtcacccatcagggcctgagctcgcccgtcacaaagagcttcaacaggggagagtgttag

SEQ ID NO: 313 - protein, 214 aa, Homo sapiens
DIQMTQSPSSLSASVGDRVTMTCRASRTISSYLSWYQQKSGKVPNLLIFGASSLQSGVPSRFSASGSGTDFTLIISSLQPEDFATYYCQQSYSSPLTFGGGTKVEIKRTVAAPSVFIFPPSDEQLKSGTASVVCLLNNFYPREAKVQWKVDNALQSGNSQESVTEQDSKDSTYSLSSTLTLSKADYEKHKVYACEVTHQGLSSPVTKSFNRGEC

SEQ ID NO: 314 - DNA, 351 bp, Homo sapiens
  source 1..351: mol_type = other DNA
gaggtgcagctggtggagtctgggggagacttggtacagcctggggggtccctgagactctcctgtacagcctctggattcatttttaggaactatgccatgaactgggtccgccaggctccagggaaggggctggagtggttgtcaggtattcttggtagtaatgataacacatactacgtagactccgtgaagggccggttcaccatttctagagacaattccaggaacacgctgtatctgcaaatgaacagcctgagagccgaggactcggccgtatattactgtgcaaaaggggacgctgggggctttgactactggggccagggaaccctggtcaccgtctcctca

SEQ ID NO: 315 - protein, 117 aa, Homo sapiens
EVQLVESGGDLVQPGGSLRLSCTASGFIFRNYAMNWVRQAPGKGLEWLSGILGSNDNTYYVDSVKGRFTISRDNSRNTLYLQMNSLRAEDSAVYYCAKGDAGGFDYWGQGTLVTVSS

SEQ ID NO: 316 - DNA, 24 bp, Homo sapiens
  source 1..24: mol_type = other DNA
ggattcatttttaggaactatgcc

SEQ ID NO: 317 - protein, 8 aa, Homo sapiens
GFIFRNYA

SEQ ID NO: 318 - DNA, 24 bp, Homo sapiens
  source 1..24: mol_type = other DNA
attcttggtagtaatgataacaca

SEQ ID NO: 319 - protein, 8 aa, Homo sapiens
ILGSNDNT

SEQ ID NO: 320 - DNA, 30 bp, Homo sapiens
  source 1..30: mol_type = other DNA
gcaaaaggggacgctgggggctttgactac

SEQ ID NO: 321 - protein, 10 aa, Homo sapiens
AKGDAGGFDY

SEQ ID NO: 322 - DNA, 336 bp, Homo sapiens
  source 1..336: mol_type = other DNA
gatgttgtgatgactcagtctccactctccctgcccgtcatccttggacagccggcctccatctcctgcaggtctagtcaaagcctcgtatccagtgatggaaacacctacttgaattggtttcagcagaggccaggccaatctccaaggcgcctaatttataaagtttctaaccgggactctggggtcccagacagattcagcggcagtgggtcaggcactgatttcacactgaaaatcagcagggtggaggctgaggatgttggggcttattactgcatgcaaggttcatactggcctccgacttttggccaggggaccaagctggagatcaaa

SEQ ID NO: 323 - protein, 112 aa, Homo sapiens
DVVMTQSPLSLPVILGQPASISCRSSQSLVSSDGNTYLNWFQQRPGQSPRRLIYKVSNRDSGVPDRFSGSGSGTDFTLKISRVEAEDVGAYYCMQGSYWPPTFGQGTKLEIK

SEQ ID NO: 324 - DNA, 33 bp, Homo sapiens
  source 1..33: mol_type = other DNA
caaagcctcgtatccagtgatggaaacacctac

SEQ ID NO: 325 - protein, 11 aa, Homo sapiens
QSLVSSDGNTY

SEQ ID NO: 326-327 - skipped (2 entries)

SEQ ID NO: 328 - DNA, 27 bp, Homo sapiens
  source 1..27: mol_type = other DNA
atgcaaggttcatactggcctccgact

SEQ ID NO: 329 - protein, 9 aa, Homo sapiens
MQGSYWPPT

SEQ ID NO: 330 - DNA, 1335 bp, Homo sapiens
  source 1..1335: mol_type = other DNA
gaggtgcagctggtggagtctgggggagacttggtacagcctggggggtccctgagactctcctgtacagcctctggattcatttttaggaactatgccatgaactgggtccgccaggctccagggaaggggctggagtggttgtcaggtattcttggtagtaatgataacacatactacgtagactccgtgaagggccggttcaccatttctagagacaattccaggaacacgctgtatctgcaaatgaacagcctgagagccgaggactcggccgtatattactgtgcaaaaggggacgctgggggctttgactactggggccagggaaccctggtcaccgtctcctcagcctccaccaagggcccatcggtcttccccctggcgccctgctccaggagcacctccgagagcacagccgccctgggctgcctggtcaaggactacttccccgaaccggtgacggtgtcgtggaactcaggcgccctgaccagcggcgtgcacaccttcccggctgtcctacagtcctcaggactctactccctcagcagcgtggtgaccgtgccctccagcagcttgggcacgaagacctacacctgcaacgtagatcacaagcccagcaacaccaaggtggacaagagagttgagtccaaatatggtcccccatgcccaccctgcccagcacctgagttcctggggggaccatcagtcttcctgttccccccaaaacccaaggacactctcatgatctcccggacccctgaggtcacgtgcgtggtggtggacgtgagccaggaagaccccgaggtccagttcaactggtacgtggatggcgtggaggtgcataatgccaagacaaagccgcgggaggagcagttcaacagcacgtaccgtgtggtcagcgtcctcaccgtcctgcaccaggactggctgaacggcaaggagtacaagtgcaaggtctccaacaaaggcctcccgtcctccatcgagaaaaccatctccaaagccaaagggcagccccgagagccacaggtgtacaccctgcccccatcccaggaggagatgaccaagaaccaggtcagcctgacctgcctggtcaaaggcttctaccccagcgacatcgccgtggagtgggagagcaatgggcagccggagaacaactacaagaccacgcctcccgtgctggactccgacggctccttcttcctctacagcaggctcaccgtggacaagagcaggtggcaggaggggaatgtcttctcatgctccgtgatgcatgaggctctgcacaaccactacacacagaagtccctctccctgtctctgggtaaatga

SEQ ID NO: 331 - protein, 444 aa, Homo sapiens
EVQLVESGGDLVQPGGSLRLSCTASGFIFRNYAMNWVRQAPGKGLEWLSGILGSNDNTYYVDSVKGRFTISRDNSRNTLYLQMNSLRAEDSAVYYCAKGDAGGFDYWGQGTLVTVSSASTKGPSVFPLAPCSRSTSESTAALGCLVKDYFPEPVTVSWNSGALTSGVHTFPAVLQSSGLYSLSSVVTVPSSSLGTKTYTCNVDHKPSNTKVDKRVESKYGPPCPPCPAPEFLGGPSVFLFPPKPKDTLMISRTPEVTCVVVDVSQEDPEVQFNWYVDGVEVHNAKTKPREEQFNSTYRVVSVLTVLHQDWLNGKEYKCKVSNKGLPSSIEKTISKAKGQPREPQVYTLPPSQEEMTKNQVSLTCLVKGFYPSDIAVEWESNGQPENNYKTTPPVLDSDGSFFLYSRLTVDKSRWQEGNVFSCSVMHEALHNHYTQKSLSLSLGK

SEQ ID NO: 332 - DNA, 660 bp, Homo sapiens
  source 1..660: mol_type = other DNA
gatgttgtgatgactcagtctccactctccctgcccgtcatccttggacagccggcctccatctcctgcaggtctagtcaaagcctcgtatccagtgatggaaacacctacttgaattggtttcagcagaggccaggccaatctccaaggcgcctaatttataaagtttctaaccgggactctggggtcccagacagattcagcggcagtgggtcaggcactgatttcacactgaaaatcagcagggtggaggctgaggatgttggggcttattactgcatgcaaggttcatactggcctccgacttttggccaggggaccaagctggagatcaaacgaactgtggctgcaccatctgtcttcatcttcccgccatctgatgagcagttgaaatctggaactgcctctgttgtgtgcctgctgaataacttctatcccagagaggccaaagtacagtggaaggtggataacgccctccaatcgggtaactcccaggagagtgtcacagagcaggacagcaaggacagcacctacagcctcagcagcaccctgacgctgagcaaagcagactacgagaaacacaaagtctacgcctgcgaagtcacccatcagggcctgagctcgcccgtcacaaagagcttcaacaggggagagtgttag

SEQ ID NO: 333 - protein, 219 aa, Homo sapiens
DVVMTQSPLSLPVILGQPASISCRSSQSLVSSDGNTYLNWFQQRPGQSPRRLIYKVSNRDSGVPDRFSGSGSGTDFTLKISRVEAEDVGAYYCMQGSYWPPTFGQGTKLEIKRTVAAPSVFIFPPSDEQLKSGTASVVCLLNNFYPREAKVQWKVDNALQSGNSQESVTEQDSKDSTYSLSSTLTLSKADYEKHKVYACEVTHQGLSSPVTKSFNRGEC

SEQ ID NO: 334 - DNA, 363 bp, Homo sapiens
  source 1..363: mol_type = other DNA
caggtgcagctggtggagtctgggggaggcgtggtcaagcctggggggtccctgagactctcctgtgcagcctctggattcaccttcagtaactctggcattcactgggtccgccaggctccaggcaaggggctggagtgggtggcacttatatcatatgctggaagtaataaatactatgcagactccgtgaagggccgattcaccatctccagagacaattccaagaacacgctgtctctgcaaatgaacagcctgagagctgaggacacggctgtgtattactgtgcgaaagaggtttggactggaacttatgattcttttgatatgtggggccgagggacaatggtcaccgtctcttca

SEQ ID NO: 335 - protein, 121 aa, Homo sapiens
QVQLVESGGGVVKPGGSLRLSCAASGFTFSNSGIHWVRQAPGKGLEWVALISYAGSNKYYADSVKGRFTISRDNSKNTLSLQMNSLRAEDTAVYYCAKEVWTGTYDSFDMWGRGTMVTVSS

SEQ ID NO: 336 - DNA, 24 bp, Homo sapiens
  source 1..24: mol_type = other DNA
ggattcaccttcagtaactctggc

SEQ ID NO: 337 - protein, 8 aa, Homo sapiens
GFTFSNSG

SEQ ID NO: 338 - DNA, 24 bp, Homo sapiens
  source 1..24: mol_type = other DNA
atatcatatgctggaagtaataaa

SEQ ID NO: 339 - protein, 8 aa, Homo sapiens
ISYAGSNK

SEQ ID NO: 340 - DNA, 42 bp, Homo sapiens
  source 1..42: mol_type = other DNA
gcgaaagaggtttggactggaacttatgattcttttgatatg

SEQ ID NO: 341 - protein, 14 aa, Homo sapiens
AKEVWTGTYDSFDM

SEQ ID NO: 342 - DNA, 1347 bp, Homo sapiens
  source 1..1347: mol_type = other DNA
caggtgcagctggtggagtctgggggaggcgtggtcaagcctggggggtccctgagactctcctgtgcagcctctggattcaccttcagtaactctggcattcactgggtccgccaggctccaggcaaggggctggagtgggtggcacttatatcatatgctggaagtaataaatactatgcagactccgtgaagggccgattcaccatctccagagacaattccaagaacacgctgtctctgcaaatgaacagcctgagagctgaggacacggctgtgtattactgtgcgaaagaggtttggactggaacttatgattcttttgatatgtggggccgagggacaatggtcaccgtctcttcagcctccaccaagggcccatcggtcttccccctggcgccctgctccaggagcacctccgagagcacagccgccctgggctgcctggtcaaggactacttccccgaaccggtgacggtgtcgtggaactcaggcgccctgaccagcggcgtgcacaccttcccggctgtcctacagtcctcaggactctactccctcagcagcgtggtgaccgtgccctccagcagcttgggcacgaagacctacacctgcaacgtagatcacaagcccagcaacaccaaggtggacaagagagttgagtccaaatatggtcccccatgcccaccctgcccagcacctgagttcctggggggaccatcagtcttcctgttccccccaaaacccaaggacactctcatgatctcccggacccctgaggtcacgtgcgtggtggtggacgtgagccaggaagaccccgaggtccagttcaactggtacgtggatggcgtggaggtgcataatgccaagacaaagccgcgggaggagcagttcaacagcacgtaccgtgtggtcagcgtcctcaccgtcctgcaccaggactggctgaacggcaaggagtacaagtgcaaggtctccaacaaaggcctcccgtcctccatcgagaaaaccatctccaaagccaaagggcagccccgagagccacaggtgtacaccctgcccccatcccaggaggagatgaccaagaaccaggtcagcctgacctgcctggtcaaaggcttctaccccagcgacatcgccgtggagtgggagagcaatgggcagccggagaacaactacaagaccacgcctcccgtgctggactccgacggctccttcttcctctacagcaggctcaccgtggacaagagcaggtggcaggaggggaatgtcttctcatgctccgtgatgcatgaggctctgcacaaccactacacacagaagtccctctccctgtctctgggtaaatga

SEQ ID NO: 343 - protein, 448 aa, Homo sapiens
QVQLVESGGGVVKPGGSLRLSCAASGFTFSNSGIHWVRQAPGKGLEWVALISYAGSNKYYADSVKGRFTISRDNSKNTLSLQMNSLRAEDTAVYYCAKEVWTGTYDSFDMWGRGTMVTVSSASTKGPSVFPLAPCSRSTSESTAALGCLVKDYFPEPVTVSWNSGALTSGVHTFPAVLQSSGLYSLSSVVTVPSSSLGTKTYTCNVDHKPSNTKVDKRVESKYGPPCPPCPAPEFLGGPSVFLFPPKPKDTLMISRTPEVTCVVVDVSQEDPEVQFNWYVDGVEVHNAKTKPREEQFNSTYRVVSVLTVLHQDWLNGKEYKCKVSNKGLPSSIEKTISKAKGQPREPQVYTLPPSQEEMTKNQVSLTCLVKGFYPSDIAVEWESNGQPENNYKTTPPVLDSDGSFFLYSRLTVDKSRWQEGNVFSCSVMHEALHNHYTQKSLSLSLGK

SEQ ID NO: 344 - DNA, 363 bp, Homo sapiens
  source 1..363: mol_type = other DNA
gaggtgcagctggtggagtctgggggaggcttggtacagcctggagggtccctgagactctcctgtgcagcctctggattcatcttcagtagttatgaaatgcattgggtccgccaggctccagggaaggggctggagtggatttcatacattagtagtagtggtactaccatatactacgcagactctgtgaagggccgattcaccatctccagagacaacgccaagaactcactgtatctgcacatgaacagcctgagagccgaggacacggctgtttattactgtacgagagcccgtataactggaactttcgatgtttttgatatctggggccaagggacaatggtcaccgtctcttca

SEQ ID NO: 345 - protein, 121 aa, Homo sapiens
EVQLVESGGGLVQPGGSLRLSCAASGFIFSSYEMHWVRQAPGKGLEWISYISSSGTTIYYADSVKGRFTISRDNAKNSLYLHMNSLRAEDTAVYYCTRARITGTFDVFDIWGQGTMVTVSS

SEQ ID NO: 346 - DNA, 24 bp, Homo sapiens
  source 1..24: mol_type = other DNA
ggattcatcttcagtagttatgaa

SEQ ID NO: 347 - protein, 8 aa, Homo sapiens
GFIFSSYE

SEQ ID NO: 348 - DNA, 24 bp, Homo sapiens
  source 1..24: mol_type = other DNA
attagtagtagtggtactaccata

SEQ ID NO: 349 - protein, 8 aa, Homo sapiens
ISSSGTTI

SEQ ID NO: 350 - DNA, 42 bp, Homo sapiens
  source 1..42: mol_type = other DNA
acgagagcccgtataactggaactttcgatgtttttgatatc

SEQ ID NO: 351 - protein, 14 aa, Homo sapiens
TRARITGTFDVFDI

SEQ ID NO: 352 - DNA, 321 bp, Homo sapiens
  source 1..321: mol_type = other DNA
gacatccagatgacccagtctccatcctccctgtctgcatctgtgggagacagagtcaccatcacttgccgggcaagtcagagcattagcagctatttaaattggtatcagcagaaaccagggaaagcccctaagctcctgatctttgctgcatccaatttacagagtggggtcccatcaaggttcagtggcagtagatctgggacagatttcactctcaccatcagcagtctgcaacctgaagattttgcaacttactactgtcaacagaattacaatatcccgtacacttttggccaggggaccaagctggagatcaaa

SEQ ID NO: 353 - protein, 107 aa, Homo sapiens
DIQMTQSPSSLSASVGDRVTITCRASQSISSYLNWYQQKPGKAPKLLIFAASNLQSGVPSRFSGSRSGTDFTLTISSLQPEDFATYYCQQNYNIPYTFGQGTKLEIK

SEQ ID NO: 354 - DNA, 27 bp, Homo sapiens
  source 1..27: mol_type = other DNA
caacagaattacaatatcccgtacact

SEQ ID NO: 355 - protein, 9 aa, Homo sapiens
QQNYNIPYT

SEQ ID NO: 356 - DNA, 1347 bp, Homo sapiens
  source 1..1347: mol_type = other DNA
gaggtgcagctggtggagtctgggggaggcttggtacagcctggagggtccctgagactctcctgtgcagcctctggattcatcttcagtagttatgaaatgcattgggtccgccaggctccagggaaggggctggagtggatttcatacattagtagtagtggtactaccatatactacgcagactctgtgaagggccgattcaccatctccagagacaacgccaagaactcactgtatctgcacatgaacagcctgagagccgaggacacggctgtttattactgtacgagagcccgtataactggaactttcgatgtttttgatatctggggccaagggacaatggtcaccgtctcttcagcctccaccaagggcccatcggtcttccccctggcgccctgctccaggagcacctccgagagcacagccgccctgggctgcctggtcaaggactacttccccgaaccggtgacggtgtcgtggaactcaggcgccctgaccagcggcgtgcacaccttcccggctgtcctacagtcctcaggactctactccctcagcagcgtggtgaccgtgccctccagcagcttgggcacgaagacctacacctgcaacgtagatcacaagcccagcaacaccaaggtggacaagagagttgagtccaaatatggtcccccatgcccaccctgcccagcacctgagttcctggggggaccatcagtcttcctgttccccccaaaacccaaggacactctcatgatctcccggacccctgaggtcacgtgcgtggtggtggacgtgagccaggaagaccccgaggtccagttcaactggtacgtggatggcgtggaggtgcataatgccaagacaaagccgcgggaggagcagttcaacagcacgtaccgtgtggtcagcgtcctcaccgtcctgcaccaggactggctgaacggcaaggagtacaagtgcaaggtctccaacaaaggcctcccgtcctccatcgagaaaaccatctccaaagccaaagggcagccccgagagccacaggtgtacaccctgcccccatcccaggaggagatgaccaagaaccaggtcagcctgacctgcctggtcaaaggcttctaccccagcgacatcgccgtggagtgggagagcaatgggcagccggagaacaactacaagaccacgcctcccgtgctggactccgacggctccttcttcctctacagcaggctcaccgtggacaagagcaggtggcaggaggggaatgtcttctcatgctccgtgatgcatgaggctctgcacaaccactacacacagaagtccctctccctgtctctgggtaaatga

SEQ ID NO: 357 - protein, 448 aa, Homo sapiens
EVQLVESGGGLVQPGGSLRLSCAASGFIFSSYEMHWVRQAPGKGLEWISYISSSGTTIYYADSVKGRFTISRDNAKNSLYLHMNSLRAEDTAVYYCTRARITGTFDVFDIWGQGTMVTVSSASTKGPSVFPLAPCSRSTSESTAALGCLVKDYFPEPVTVSWNSGALTSGVHTFPAVLQSSGLYSLSSVVTVPSSSLGTKTYTCNVDHKPSNTKVDKRVESKYGPPCPPCPAPEFLGGPSVFLFPPKPKDTLMISRTPEVTCVVVDVSQEDPEVQFNWYVDGVEVHNAKTKPREEQFNSTYRVVSVLTVLHQDWLNGKEYKCKVSNKGLPSSIEKTISKAKGQPREPQVYTLPPSQEEMTKNQVSLTCLVKGFYPSDIAVEWESNGQPENNYKTTPPVLDSDGSFFLYSRLTVDKSRWQEGNVFSCSVMHEALHNHYTQKSLSLSLGK

SEQ ID NO: 358 - DNA, 645 bp, Homo sapiens
  source 1..645: mol_type = other DNA
gacatccagatgacccagtctccatcctccctgtctgcatctgtgggagacagagtcaccatcacttgccgggcaagtcagagcattagcagctatttaaattggtatcagcagaaaccagggaaagcccctaagctcctgatctttgctgcatccaatttacagagtggggtcccatcaaggttcagtggcagtagatctgggacagatttcactctcaccatcagcagtctgcaacctgaagattttgcaacttactactgtcaacagaattacaatatcccgtacacttttggccaggggaccaagctggagatcaaacgaactgtggctgcaccatctgtcttcatcttcccgccatctgatgagcagttgaaatctggaactgcctctgttgtgtgcctgctgaataacttctatcccagagaggccaaagtacagtggaaggtggataacgccctccaatcgggtaactcccaggagagtgtcacagagcaggacagcaaggacagcacctacagcctcagcagcaccctgacgctgagcaaagcagactacgagaaacacaaagtctacgcctgcgaagtcacccatcagggcctgagctcgcccgtcacaaagagcttcaacaggggagagtgttag

SEQ ID NO: 359 - protein, 214 aa, Homo sapiens
DIQMTQSPSSLSASVGDRVTITCRASQSISSYLNWYQQKPGKAPKLLIFAASNLQSGVPSRFSGSRSGTDFTLTISSLQPEDFATYYCQQNYNIPYTFGQGTKLEIKRTVAAPSVFIFPPSDEQLKSGTASVVCLLNNFYPREAKVQWKVDNALQSGNSQESVTEQDSKDSTYSLSSTLTLSKADYEKHKVYACEVTHQGLSSPVTKSFNRGEC

SEQ ID NO: 360 - DNA, 366 bp, Homo sapiens
  source 1..366: mol_type = other DNA
caggtgcagctgcaggagtcgggcccaggactggtgaagccttcacagaccctgtccctcacctgtactgtctctggtggctccatcaccagtggcggttactactggagctggatccgccagtacccagggcagggcctggagtggattggttacatctattatagtgggaagacctactacaatccgtcttttacgagtcgaattaccatatcagtagacacgtctaagaagcagttctccctgaagatgagctctgtgactgccgcggacacggccgtgtattattgtgcgagagcgggattcacctctagtaacggctggttcgacccctggggccagggaaccctggtcaccgtctcctca

SEQ ID NO: 361 - protein, 122 aa, Homo sapiens
QVQLQESGPGLVKPSQTLSLTCTVSGGSITSGGYYWSWIRQYPGQGLEWIGYIYYSGKTYYNPSFTSRITISVDTSKKQFSLKMSSVTAADTAVYYCARAGFTSSNGWFDPWGQGTLVTVSS

SEQ ID NO: 362 - DNA, 30 bp, Homo sapiens
  source 1..30: mol_type = other DNA
ggtggctccatcaccagtggcggttactac

SEQ ID NO: 363 - protein, 10 aa, Homo sapiens
GGSITSGGYY

SEQ ID NO: 364 - DNA, 21 bp, Homo sapiens
  source 1..21: mol_type = other DNA
atctattatagtgggaagacc

SEQ ID NO: 365 - DNA, 42 bp, Homo sapiens
  source 1..42: mol_type = other DNA
gcgagagcgggattcacctctagtaacggctggttcgacccc

SEQ ID NO: 366 - protein, 14 aa, Homo sapiens
ARAGFTSSNGWFDP

SEQ ID NO: 367 - DNA, 321 bp, Homo sapiens
  source 1..321: mol_type = other DNA
gacatccagatgacccagtctccatcctccctatctgcatctgtaggagacagagtcaccatcacttgccgggcaagtcagaacattcgcagctatttgaattggtatcagcagaaaccagggaaagccccaaaactcctgatctattctgcatccagtttgcaaagtggggtcccatcaaggttcagtggcagtggatctgggacagatttcactctcaccatcagcagtctgcaacctgaagattttccaacttactactgtcaacagacttacagttccccgtggacgttcggccctgggaccaaggtggaaatcaaa

SEQ ID NO: 368 - protein, 107 aa, Homo sapiens
DIQMTQSPSSLSASVGDRVTITCRASQNIRSYLNWYQQKPGKAPKLLIYSASSLQSGVPSRFSGSGSGTDFTLTISSLQPEDFPTYYCQQTYSSPWTFGPGTKVEIK

SEQ ID NO: 369 - DNA, 18 bp, Homo sapiens
  source 1..18: mol_type = other DNA
cagaacattcgcagctat

SEQ ID NO: 370 - protein, 6 aa, Homo sapiens
QNIRSY

SEQ ID NO: 371-372 - skipped (2 entries)

SEQ ID NO: 373 - DNA, 27 bp, Homo sapiens
  source 1..27: mol_type = other DNA
caacagacttacagttccccgtggacg

SEQ ID NO: 374 - protein, 9 aa, Homo sapiens
QQTYSSPWT

SEQ ID NO: 375 - DNA, 1350 bp, Homo sapiens
  source 1..1350: mol_type = other DNA
caggtgcagctgcaggagtcgggcccaggactggtgaagccttcacagaccctgtccctcacctgtactgtctctggtggctccatcaccagtggcggttactactggagctggatccgccagtacccagggcagggcctggagtggattggttacatctattatagtgggaagacctactacaatccgtcttttacgagtcgaattaccatatcagtagacacgtctaagaagcagttctccctgaagatgagctctgtgactgccgcggacacggccgtgtattattgtgcgagagcgggattcacctctagtaacggctggttcgacccctggggccagggaaccctggtcaccgtctcctcagcctccaccaagggcccatcggtcttccccctggcgccctgctccaggagcacctccgagagcacagccgccctgggctgcctggtcaaggactacttccccgaaccggtgacggtgtcgtggaactcaggcgccctgaccagcggcgtgcacaccttcccggctgtcctacagtcctcaggactctactccctcagcagcgtggtgaccgtgccctccagcagcttgggcacgaagacctacacctgcaacgtagatcacaagcccagcaacaccaaggtggacaagagagttgagtccaaatatggtcccccatgcccaccctgcccagcacctgagttcctggggggaccatcagtcttcctgttccccccaaaacccaaggacactctcatgatctcccggacccctgaggtcacgtgcgtggtggtggacgtgagccaggaagaccccgaggtccagttcaactggtacgtggatggcgtggaggtgcataatgccaagacaaagccgcgggaggagcagttcaacagcacgtaccgtgtggtcagcgtcctcaccgtcctgcaccaggactggctgaacggcaaggagtacaagtgcaaggtctccaacaaaggcctcccgtcctccatcgagaaaaccatctccaaagccaaagggcagccccgagagccacaggtgtacaccctgcccccatcccaggaggagatgaccaagaaccaggtcagcctgacctgcctggtcaaaggcttctaccccagcgacatcgccgtggagtgggagagcaatgggcagccggagaacaactacaagaccacgcctcccgtgctggactccgacggctccttcttcctctacagcaggctcaccgtggacaagagcaggtggcaggaggggaatgtcttctcatgctccgtgatgcatgaggctctgcacaaccactacacacagaagtccctctccctgtctctgggtaaatga

SEQ ID NO: 376 - protein, 449 aa, Homo sapiens
QVQLQESGPGLVKPSQTLSLTCTVSGGSITSGGYYWSWIRQYPGQGLEWIGYIYYSGKTYYNPSFTSRITISVDTSKKQFSLKMSSVTAADTAVYYCARAGFTSSNGWFDPWGQGTLVTVSSASTKGPSVFPLAPCSRSTSESTAALGCLVKDYFPEPVTVSWNSGALTSGVHTFPAVLQSSGLYSLSSVVTVPSSSLGTKTYTCNVDHKPSNTKVDKRVESKYGPPCPPCPAPEFLGGPSVFLFPPKPKDTLMISRTPEVTCVVVDVSQEDPEVQFNWYVDGVEVHNAKTKPREEQFNSTYRVVSVLTVLHQDWLNGKEYKCKVSNKGLPSSIEKTISKAKGQPREPQVYTLPPSQEEMTKNQVSLTCLVKGFYPSDIAVEWESNGQPENNYKTTPPVLDSDGSFFLYSRLTVDKSRWQEGNVFSCSVMHEALHNHYTQKSLSLSLGK

SEQ ID NO: 377 - DNA, 645 bp, Homo sapiens
  source 1..645: mol_type = other DNA
gacatccagatgacccagtctccatcctccctatctgcatctgtaggagacagagtcaccatcacttgccgggcaagtcagaacattcgcagctatttgaattggtatcagcagaaaccagggaaagccccaaaactcctgatctattctgcatccagtttgcaaagtggggtcccatcaaggttcagtggcagtggatctgggacagatttcactctcaccatcagcagtctgcaacctgaagattttccaacttactactgtcaacagacttacagttccccgtggacgttcggccctgggaccaaggtggaaatcaaacgaactgtggctgcaccatctgtcttcatcttcccgccatctgatgagcagttgaaatctggaactgcctctgttgtgtgcctgctgaataacttctatcccagagaggccaaagtacagtggaaggtggataacgccctccaatcgggtaactcccaggagagtgtcacagagcaggacagcaaggacagcacctacagcctcagcagcaccctgacgctgagcaaagcagactacgagaaacacaaagtctacgcctgcgaagtcacccatcagggcctgagctcgcccgtcacaaagagcttcaacaggggagagtgttag

SEQ ID NO: 378 - protein, 214 aa, Homo sapiens
DIQMTQSPSSLSASVGDRVTITCRASQNIRSYLNWYQQKPGKAPKLLIYSASSLQSGVPSRFSGSGSGTDFTLTISSLQPEDFPTYYCQQTYSSPWTFGPGTKVEIKRTVAAPSVFIFPPSDEQLKSGTASVVCLLNNFYPREAKVQWKVDNALQSGNSQESVTEQDSKDSTYSLSSTLTLSKADYEKHKVYACEVTHQGLSSPVTKSFNRGEC

SEQ ID NO: 379 - protein, 268 aa, synthetic construct
  REGION 1..268: note = Human IL2R extracellular domain expressed with a C-terminal myc-myc-hexahistidine tag
LNTTILTPNGNEDTTADFFLTTMPTDSLSVSTLPLPEVQCFVFNVEYMNCTWNSSSEPQPTNLTLHYWYKNSDNDKVQKCSHYLFSEEITSGCQLQKKEIHLYQTFVVQLQDPREPRRQATQMLKLQNLVIPWAPENLTLHKLSESQLELNWNNRFLNHCLEHLVQYRTDWDHSWTEQSVDYRHKFSLPSVDGQKRYTFRVRSRFNPLCGSAQHWSEWSHPIHWGSNTSKENPFLFALEAEQKLISEEDLGGEQKLISEEDLHHHHHH

SEQ ID NO: 380 - protein, 268 aa, synthetic construct
  REGION 1..268: note = Macaca fascicularis IL2R extracellular domain expressed with a C-terminal myc-myc-hexahistidine tag
LNTTILTPNGNEDATTDFFLTSMPTDSLSVSTLPLPEVQCFVFNVEYMNCTWNSSSEPQPTNLTLHYWYKNSDNDKVQKCSHYLFSEEITSGCQLQKKEIHLYQTFVVQLQDPREPRRQATQMLKLQNLVIPWAPENLTLRKLSESQLELNWNNRFLNHCLEHLVQYRTDWDHSWTEQSVDYRHKFSLPSVDGQKRYTFRVRSRFNPLCGSAQHWSEWSHPIHWGSNSSKENPFLFALEAEQKLISEEDLGGEQKLISEEDLHHHHHH

SEQ ID NO: 381 - protein, 473 aa, synthetic construct
  REGION 1..473: note = Human IL2R extracellular domain expressed with a C-terminal mouse IgG2a Fc tag
LNTTILTPNGNEDTTADFFLTTMPTDSLSVSTLPLPEVQCFVFNVEYMNCTWNSSSEPQPTNLTLHYWYKNSDNDKVQKCSHYLFSEEITSGCQLQKKEIHLYQTFVVQLQDPREPRRQATQMLKLQNLVIPWAPENLTLHKLSESQLELNWNNRFLNHCLEHLVQYRTDWDHSWTEQSVDYRHKFSLPSVDGQKRYTFRVRSRFNPLCGSAQHWSEWSHPIHWGSNTSKENPFLFALEAEPRGPTIKPCPPCKCPAPNLLGGPSVFIFPPKIKDVLMISLSPIVTCVVVDVSEDDPDVQISWFVNNVEVHTAQTQTHREDYNSTLRVVSALPIQHQDWMSGKEFKCKVNNKDLPAPIERTISKPKGSVRAPQVYVLPPPEEEMTKKQVTLTCMVTDFMPEDIYVEWTNNGKTELNYKNTEPVLDSDGSYFMYSKLRVEKKNWVERNSYSCSVVHEGLHNHHTTKSFSRTPGK

SEQ ID NO: 382 - protein, 159 aa, synthetic construct
  REGION 1..159: note = D1 domain of human IL-2R extracellular domain expressed with a C-terminal myc-myc-hexahistidine tag
LNTTILTPNGNEDTTADFFLTTMPTDSLSVSTLPLPEVQCFVFNVEYMNCTWNSSSEPQPTNLTLHYWYKNSDNDKVQKCSHYLFSEEITSGCQLQKKEIHLYQTFVVQLQDPREPRRQATQMLKLQNLVIEQKLISEEDLGGEQKLISEEDLHHHHHH

SEQ ID NO: 383 - protein, 116 aa, synthetic construct
  REGION 1..116: note = D2 domain of human IL2R extracellular domain expressed with a C-terminal myc-myc-hexahistidine tag
PWAPENLTLHKLSESQLELNWNNRFLNHCLEHLVQYRTDWDHSWTEQSVDYRHKFSLPSVDGQKRYTFRVRSRFNPLCGSAQHWSEWSEQKLISEEDLGGEQKLISEEDLHHHHHH

SEQ ID NO: 384 - protein, 269 aa, synthetic construct
  REGION 1..269: note = Mouse IL2R extracellular domain expressed with a C-terminal myc-myc-hexahistidine tag
WSSKVLMSSANEDIKADLILTSTAPEHLSAPTLPLPEVQCFVFNIEYMNCTWNSSSEPQATNLTLHYRYKVSDNNTFQECSHYLFSKEITSGCQIQKEDIQLYQTFVVQLQDPQKPQRRAVQKLNLQNLVIPRAPENLTLSNLSESQLELRWKSRHIKERCLQYLVQYRSNRDRSWTELIVNHEPRFSLPSVDELKRYTFRVRSRYNPICGSSQQWSKWSQPVHWGSHTVEENPSLFALEAEQKLISEEDLGGEQKLISEEDLHHHHHH

SEQ ID NO: 385 - protein, 268 aa, synthetic construct
  REGION 1..268: note = Rat IL2R extracellular domain expressed with a C-terminal myc-myc-hexahistidine tag
WSSKVLMSSGNEDTKSDLLLTSMDLKHLSVPTLPLPEVQCFVFNVEYMNCTWNSSSEPQPTNLTMHYRYKGSDNNTFQECSHYLFSKEITSGCQIQKEDIQLYQTFVVQLQDPQKPQRRAEQKLNLQNLVIPWAPENLTLYNLSESQVELRWKSRYIERCLQYLVQYRSNRDRSWTEQIVDHEPRFSLPSVDEQKLYTFRVRSRFNPICGSTQQWSKWSQPIHWGSHTAEENPSLFALEAEQKLISEEDLGGEQKLISEEDLHHHHHH

SEQ ID NO: 386 - protein, 5 aa, synthetic construct
  REGION 1..5: note = G4S linker
GGGGS